European Patent Specification EP 3 461 890 B1, published September 24, 2025. Title: Total fermentation of oligosaccharides. Applicant: Jennewein Biotechnologie GmbH. The sequence listing filed with the application follows.

SEQUENCE LISTING (34 sequences)

SEQ ID NO: 1 - DNA, 2851 bp, Artificial Sequence
  Ptet-lacY-FRT-aadA-FRT
tggccagatgattaattcctaatttttgttgacactctatcattgatagagttattttaccactccctatcagtgatagagaaaagtgaaatgaatagttcgacaaaaatctagaaataattttgtttaactttaagaaggagatatacaaatgtactatttaaaaaacacaaacttttggatgttcggtttattctttttcttttacttttttatcatgggagcctacttcccgtttttcccgatttggctacatgacatcaaccatatcagcaaaagtgatacgggtattatttttgccgctatttctctgttctcgctattattccaaccgctgtttggtctgctttctgacaaactcgggctgcgcaaatacctgctgtggattattaccggcatgttagtgatgtttgcgccgttctttatttttatcttcgggccactgttacaatacaacattttagtaggatcgattgttggtggtatttatctaggcttttgttttaacgccggtgcgccagcagtagaggcatttattgagaaagtcagccgtcgcagtaatttcgaatttggtcgcgcgcggatgtttggctgtgttggctgggcgctgtgtgcctcgattgtcggcatcatgttcaccatcaataatcagtttgttttctggctgggctctggctgtgcactcatcctcgccgttttactctttttcgccaaaacggatgcgccctcttctgccacggttgccaatgcggtaggtgccaaccattcggcatttagccttaagctggcactggaactgttcagacagccaaaactgtggtttttgtcactgtatgttattggcgtttcctgcacctacgatgtttttgaccaacagtttgctaatttctttacttcgttctttgctaccggtgaacagggtacgcgggtatttggctacgtaacgacaatgggcgaattacttaacgcctcgattatgttctttgcgccactgatcattaatcgcatcggtgggaaaaacgccctgctgctggctggcactattatgtctgtacgtattattggctcatcgttcgccacctcagcgctggaagtggttattctgaaaacgctgcatatgtttgaagtaccgttcctgctggtgggctgctttaaatatattaccagccagtttgaagtgcgtttttcagcgacgatttatctggtctgtttctgcttctttaagcaactggcgatgatttttatgtctgtactggcgggcaatatgtatgaaagcatcggtttccagggcgcttatctggtgctgggtctggtggcgctgggcttcaccttaatttccgtgttcacgcttagcggccccggcccgctttccctgctgcgtcgtcaggtgaatgaagtcgctgggagctaagcggccgcgtcgacacgcaaaaaggccatccgtcaggatggccttctgcttaatttgatgcctggcagtttatggcgggcgtcctgcccgccaccctccgggccgttgcttcgcaacgttcaaatccgctcccggcggatttgtcctactcaggagagcgttcaccgacaaacaacagataaaacgaaaggcccagtctttcgactgagcctttcgttttatttgatgcctggcagttccctactctcgcatggggagaccccacactaccatcatgtatgaatatcctccttagttcctattccgaagttcctattctctagaaagtataggaacttcggcgcgtcctacctgtgacacgcgtgccgcagtctcacgcccggagcgtagcgaccgagtgagctagctatttgtttatttttctaaatacattcaaatatgtatccgctcatgagacaataaccctgataaatgcttcaataatattgaaaaaggaagagtatgagggaagcggtgatcgccgaagtatcgactcaactatcagaggtagttggcgtcatcgagcgccatctcgaaccgacgttgctggccgtacatttgtacggctccgcagtggatggcggcctgaagccacacagtgatattgatttgctggttacggtgaccgtaaggcttgatgaaacaacgcggcgagctttgatcaacgaccttttggaaacttcggcttcccctggagagagcgagattctccgcgctgtagaagtcaccattgttgtgcacgacgacatcattccgtggcgttatccagctaagcgcgaactgcaatttggagaatggcagcgcaatgacattcttgcaggtatcttcgagccagccacgatcgacattgatctggctatcttgctgacaaaagcaagagaacatagcgttgccttggtaggtccagcggcggaggaactctttgatccggttcctgaacaggatctatttgaggcgctaaatgaaaccttaacgctatggaactcgccgcccgactgggctggcgatgagcgaaatgtagtgcttacgttgtcccgcatttggtacagcgcagtaaccggcaaaatcgcgccgaaggatgtcgctgccgactgggcaatggagcgcctgccggcccagtatcagcccgtcatacttgaagctagacaggcttatcttggacaagaagaagatcgcttggcctcgcgcgcagatcagttggaagaatttgtccactacgtgaaaggcgagatcaccaaggtagtcggcaaataatgtctaacaattcgttcaagccgaggggccgcaagatccggccacgatgacccggtcgtcgggtaccggcagggcggggcgtaaggcgcgccatttaaatgaagttcctattccgaagttcctattctctagaaagtataggaactt

SEQ ID NO: 2 - DNA, 2858 bp, Artificial Sequence
  Ptet-wbgL-FRT-neo-FRT
ggccagatgattaattcctaatttttgttgacactctatcattgatagagttattttaccactccctatcagtgatagagaaaagtgaaatgaatagttcgacaaaaatctagaaataattttgtttaactttaagaaggagatatacaaatgggcagcattattcgtctgcagggtggtctgggtaatcagctgtttcagtttagctttggttatgccctgagcaaaattaatggtacaccgctgtatttcgacattagccattatgccgaaaacgatgatcatggtggttatcgtctgaataatctgcagattccggaagaatatctgcagtattataccccgaaaattaataatatttataaactgctggtgcgtggcagccgtctgtatccggatatttttctgtttctgggcttttgcaacgaatttcatgcctatggctacgattttgaatatattgcccagaaatggaaaagcaaaaaatacattggctactggcagagcgaacacttttttcataaacatattctggacctgaaagaattttttattccgaaaaatgtgagcgaacaggcaaatctgctggcagcaaaaattctggaaagccagagcagcctgagcattcatattcgtcgtggcgattatattaaaaacaaaaccgcaaccctgacacatggtgtttgtagcctggaatattataaaaaagccctgaacaaaatccgcgatctggcaatgattcgtgatgtgtttatctttagcgacgatatcttctggtgcaaagaaaatattgaaaccctgctgagcaaaaaatataatatttattatagcgaagatctgagccaagaagaggatctgtggctgatgagcctggcaaatcatcatattattgccaatagcagctttagttggtggggtgcatatctgggtagcagcgcaagccagattgttatttatccgaccccgtggtatgatattaccccgaaaaacacctatatcccgattgtgaaccattggatcaacgttgataaacatagcagctgctaagcggccgcgtcgacacgcaaaaaggccatccgtcaggatggccttctgcttaatttgatgcctggcagtttatggcgggcgtcctgcccgccaccctccgggccgttgcttcgcaacgttcaaatccgctcccggcggatttgtcctactcaggagagcgttcaccgacaaacaacagataaaacgaaaggcccagtctttcgactgagcctttcgttttatttgatgcctggcagttccctactctcgcatggggagaccccacactaccatcatgtatgaatatcctccttagttcctattccgaagttcctattctctagaaagtataggaacttcggcgcgtcctacctgtgacacgcgtcaagatcccctcacgctgccgcaagcactcagggcgcaagggctgctaaaggaagcggaacacgtagaaagccagtccgcagaaacggtgctgaccccggatgaatgtcagctactgggctatctggacaagggaaaacgcaagcgcaaagagaaagcaggtagcttgcagtgggcttacatggcgatagctagactgggcggttttatggacagcaagcgaaccggaattgccagctggggcgccctctggtaaggttgggaagccctgcaaagtaaactggatggctttcttgccgccaaggatctgatggcgcaggggatcaagatctgatcaagagacaggatgaggatcgtttcgcatgattgaacaagatggattgcacgcaggttctccggccgcttgggtggagaggctattcggctatgactgggcacaacagacaatcggctgctctgatgccgccgtgttccggctgtcagcgcaggggcgcccggttctttttgtcaagaccgacctgtccggtgccctgaatgaactgcaggacgaggcagcgcggctatcgtggctggccacgacgggcgttccttgcgcagctgtgctcgacgttgtcactgaagcgggaagggactggctgctattgggcgaagtgccggggcaggatctcctgtcatctcaccttgctcctgccgagaaagtatccatcatggctgatgcaatgcggcggctgcatacgcttgatccggctacctgcccattcgaccaccaagcgaaacatcgcatcgagcgagcacgtactcggatggaagccggtcttgtcgatcaggatgatctggacgaagagcatcaggggctcgcgccagccgaactgttcgccaggctcaaggcgcgcatgcccgacggcgaggatctcgtcgtgacccatggcgatgcctgcttgccgaatatcatggtggaaaatggccgcttttctggattcatcgactgtggccggctgggtgtggcggaccgctatcaggacatagcgttggctacccgtgatattgctgaagagcttggcggcgaatgggctgaccgcttcctcgtgctttacggtatcgccgctcccgattcgcagcgcatcgccttctatcgccttcttgacgagttcttctgagcgggactctggggttcgaaatgaccgaccaagcgacgcccaacctgccatcacgagatttcgattccaccgccgccttctatgaaaggttgggcttcggaatcgttttccgggacgccggctggatgatcctccagcgcggggatctcatgctggagttcttcgcccaccccagcttcaaaagcgctctcggtaccggcagggcggggcgtaaggcgcgccatttaaatgaagttcctattccgaagttcctattctctagaaagtataggaacttcgaagcagctccag

SEQ ID NO: 3 - DNA, 2631 bp, Artificial Sequence
  Ptet-yberc0001_9420-FRT-cat-FRT
ggccagatgattaattcctaatttttgttgacactctatcattgatagagttattttaccactccctatcagtgatagagaaaagtgaaatgaatagttcgacaaaaatctagaaataattttgtttaactttaagaaggagatatacaaatgaagtcggcactgaccttttcccgtcgcatcaatccggtgtttctggcgttctttgtcgttgcttttctgagcggtatcgcaggcgcactgcaggctccgaccctgagtctgtttctgtccacggaagtgaaagttcgtccgctgtgggttggtctgttctataccgtcaacgcaatcgctggcattacggttagctttatcctggcgaaacgttcagattcgcgcggtgaccgtcgcaagctgattatggtgtgctatctgatggcggttggcaactgtctgctgtttgccttcaatcgtgattacctgaccctgatcacggcaggtgtgctgctggcgagcgttgccaacaccgcaatgccgcagattttcgcgctggcccgtgaatatgccgacagctctgcacgcgaagtggttatgtttagttccatcatgcgcgctcaactgagtctggcatgggtgattggtccgccgctgtcctttatgctggcgctgaattacggttttaccctgatgttctcaatcgcggccggcattttcgttctgtcggccctggtcgtgtggtttatcctgccgagtgtcccgcgtgcagaaccggttgtcgatgcaccggtggttgtccagggttcactgttcgcagacaaaaacgttctgctgctgtttatcgcgtcgatgctgatgtggacctgcaatacgatgtatattatcgatatgccgctgtacattaccgcaagcctgggtctgccggaacgtctggctggtctgctgatgggtaccgcagctggcctggaaattccgatcatgctgctggcgggttattctgtgcgttactttggcaaacgcaagattatgctgttcgctgttctggcgggtgtcctgttttataccggcctggttctgtttaaattcaagacggccctgatgctgctgcagatctttaacgcaattttcatcggtattgtggctggcattggtatgctgtacttccaagatctgatgccgggtcgtgcaggtgcagcaaccacgctgtttaccaatagcatctctacgggtgtcattctggcaggcgtgctgcaaggcggtctgaccgaaacgtggggccatgacagcgtctatgtgatggcgatggtcctgtctattctggccctgattatctgtgcacgtgtgcgcgaagcttaaatcgatactagcataaccccttggggcctctaaacgcgtcgacacgcaaaaaggccatccgtcaggatggccttctgcttaatttgatgcctggcagtttatggcgggcgtcctgcccgccaccctccgggccgttgcttcgcaacgttcaaatccgctcccggcggatttgtcctactcaggagagcgttcaccgacaaacaacagataaaacgaaaggcccagtctttcgactgagcctttcgttttatttgatgcctggcagttccctactctcgcatggggagaccccacactaccatcatgtatgaatatcctccttagttcctattccgaagttcctattctctagaaagtataggaacttcggcgcgtcctacctgtgacggaagatcacttcgcagaataaataaatcctggtgtccctgttgataccgggaagccctgggccaacttttggcgaaaatgagacgttgatcggcacgtaagaggttccaactttcaccataatgaaataagatcactaccgggcgtattttttgagttgtcgagattttcaggagctaaggaagctaaaatggagaaaaaaatcactggatataccaccgttgatatatcccaatggcatcgtaaagaacattttgaggcatttcagtcagttgctcaatgtacctataaccagaccgttcagctggatattacggcctttttaaagaccgtaaagaaaaataagcacaagttttatccggcctttattcacattcttgcccgcctgatgaatgctcatccggaattacgtatggcaatgaaagacggtgagctggtgatatgggatagtgttcacccttgttacaccgttttccatgagcaaactgaaacgttttcatcgctctggagtgaataccacgacgatttccggcagtttctacacatatattcgcaagatgtggcgtgttacggtgaaaacctggcctatttccctaaagggtttattgagaatatgtttttcgtctcagccaatccctgggtgagtttcaccagttttgatttaaacgtggccaatatggacaacttcttcgcccccgttttcaccatgggcaaatattatacgcaaggcgacaaggtgctgatgccgctggcgattcaggttcatcatgccgtttgtgatggcttccatgtcggcagatgcttaatgaatacaacagtactgcgatgagtggcagggcggggcgtaaggcgcgccatttaaatgaagttcctattccgaagttcctattctctagaaagtataggaacttc

SEQ ID NO: 4 - DNA, 6783 bp, Artificial Sequence
  Ptet-manCB,PT5-gmd-wcaG-FRT-dhfr-FRT
gccagatgattaattcctaatttttgttgacactctatcattgatagagttattttaccactccctatcagtgatagagaaaagtgaaatgaatagttcgacaaaaatctagaaataattttgtttaactttaagaaggagatatacaatttcgtcgacacacaggaaacatattaaaaattaaaacctgcaggagtttgaaggagatagaaccatggcgcagtcgaaactctatccagttgtgatggcaggtggctccggtagccgcttatggccgctttcccgcgtactttatcccaagcagtttttatgcctgaaaggcgatctcaccatgctgcaaaccaccatctgccgcctgaacggcgtggagtgcgaaagcccggtggtgatttgcaatgagcagcaccgctttattgtcgcggaacagctgcgtcaactgaacaaacttaccgagaacattattctcgaaccggcagggcgaaacacggcacctgccattgcgctggcggcgctggcggcaaaacgtcatagcccggagagcgacccgttaatgctggtattggcggcggatcatgtgattgccgatgaagacgcgttccgtgccgccgtgcgtaatgccatgccatatgccgaagcgggcaagctggtgaccttcggcattgtgccggatctaccagaaaccggttatggctatattcgtcgcggtgaagtgtctgcgggtgagcaggatatggtggcctttgaagtggcgcagtttgtcgaaaaaccgaatctggaaaccgctcaggcctatgtggcaagcggcgaatattactggaacagcggtatgttcctgttccgcgccggacgctatctcgaagaactgaaaaaatatcgcccggatatcctcgatgcctgtgaaaaagcgatgagcgccgtcgatccggatctcaattttattcgcgtggatgaagaagcgtttctcgcctgcccggaagagtcggtggattacgcggtcatggaacgtacggcagatgctgttgtggtgccgatggatgcgggctggagcgatgttggctcctggtcttcattatgggagatcagcgcccacaccgccgagggcaacgtttgccacggcgatgtgattaatcacaaaactgaaaacagctatgtgtatgctgaatctggcctggtcaccaccgtcggggtgaaagatctggtagtggtgcagaccaaagatgcggtgctgattgccgaccgtaacgcggtacaggatgtgaaaaaagtggtcgagcagatcaaagccgatggtcgccatgagcatcgggtgcatcgcgaagtgtatcgtccgtggggcaaatatgactctatcgacgcgggcgaccgctaccaggtgaaacgcatcaccgtgaaaccgggcgagggcttgtcggtacagatgcaccatcaccgcgcggaacactgggtggttgtcgcgggaacggcaaaagtcaccattgatggtgatatcaaactgcttggtgaaaacgagtccatttatattccgctgggggcgacgcattgcctggaaaacccggggaaaattccgctcgatttaattgaagtgcgctccggctcttatctcgaagaggatgatgtggtgcgtttcgcggatcgctacggacgggtgtaaacgtcgcatcaggcaatgaatgcgaaaccgcggtgtaaataacgacaaaaataaaattggccgcttcggtcagggccaactattgcctgaaaaagggtaacgatatgaaaaaattaacctgctttaaagcctatgatattcgcgggaaattaggcgaagaactgaatgaagatatcgcctggcgcattggtcgcgcctatggcgaatttctcaaaccgaaaaccattgtgttaggcggtgatgtccgcctcaccagcgaaaccttaaaactggcgctggcgaaaggtttacaggatgcgggcgttgacgtgctggatattggtatgtccggcaccgaagagatctatttcgccacgttccatctcggcgtggatggcggcattgaagttaccgccagccataatccgatggattataacggcatgaagctggttcgcgagggggctcgcccgatcagcggagataccggactgcgcgacgtccagcgtctggctgaagccaacgactttcctcccgtcgatgaaaccaaacgcggtcgctatcagcaaatcaacctgcgtgacgcttacgttgatcacctgttcggttatatcaatgtcaaaaacctcacgccgctcaagctggtgatcaactccgggaacggcgcagcgggtccggtggtggacgccattgaagcccgctttaaagccctcggcgcgcccgtggaattaatcaaagtgcacaacacgccggacggcaatttccccaacggtattcctaacccactactgccggaatgccgcgacgacacccgcaatgcggtcatcaaacacggcgcggatatgggcattgcttttgatggcgattttgaccgctgtttcctgtttgacgaaaaagggcagtttattgagggctactacattgtcggcctgttggcagaagcattcctcgaaaaaaatcccggcgcgaagatcatccacgatccacgtctctcctggaacaccgttgatgtggtgactgccgcaggtggcacgccggtaatgtcgaaaaccggacacgcctttattaaagaacgtatgcgcaaggaagacgccatctatggtggcgaaatgagcgcccaccattacttccgtgatttcgcttactgcgacagcggcatgatcccgtggctgctggtcgccgaactggtgtgcctgaaagataaaacgctgggcgaactggtacgcgaccggatggcggcgtttccggcaagcggtgagatcaacagcaaactggcgcaacccgttgaggcgattaaccgcgtggaacagcattttagccgtgaggcgctggcggtggatcgcaccgatggcatcagcatgacctttgccgactggcgctttaacctgcgcacctccaataccgaaccggtggtgcgcctgaatgtggaatcgcgcggtgatgtgccgctgatggaagcgcgaacgcgaactctgctgacgttgctgaacgagtaaaaacgcggccgcgatatcgttgtaaaacgacggccagtgcaagaatcataaaaaatttatttgctttcaggaaaatttttctgtataatagattcataaatttgagagaggagtttttgtgagcggataacaattccccatcttagtatattagttaagtataaatacaccgcggaggacgaaggagatagaaccatgtcaaaagtcgctctcatcaccggtgtaaccggacaagacggttcttacctggcagagtttctgctggaaaaaggttacgaggtgcatggtattaagcgtcgcgcatcgtcattcaacaccgagcgcgtggatcacatttatcaggatccgcacacctgcaacccgaaattccatctgcattatggcgacctgagtgatacctctaacctgacgcgcattttgcgtgaagtacagccggatgaagtgtacaacctgggcgcaatgagccacgttgcggtctcttttgagtcaccagaatataccgctgacgtcgacgcgatgggtacgctgcgcctgctggaggcgatccgcttcctcggtctggaaaagaaaactcgtttctatcaggcttccacctctgaactgtatggtctggtgcaggaaattccgcagaaagagaccacgccgttctacccgcgatctccgtatgcggtcgccaaactgtacgcctactggatcaccgttaactaccgtgaatcctacggcatgtacgcctgtaacggaattctcttcaaccatgaatccccgcgccgcggcgaaaccttcgttacccgcaaaatcacccgcgcaatcgccaacatcgcccaggggctggagtcgtgcctgtacctcggcaatatggattccctgcgtgactggggccacgccaaagactacgtaaaaatgcagtggatgatgctgcagcaggaacagccggaagatttcgttatcgcgaccggcgttcagtactccgtgcgtcagttcgtggaaatggcggcagcacagctgggcatcaaactgcgctttgaaggcacgggcgttgaagagaagggcattgtggtttccgtcaccgggcatgacgcgccgggcgttaaaccgggtgatgtgattatcgctgttgacccgcgttacttccgtccggctgaagttgaaacgctgctcggcgacccgaccaaagcgcacgaaaaactgggctggaaaccggaaatcaccctcagagagatggtgtctgaaatggtggctaatgacctcgaagcggcgaaaaaacactctctgctgaaatctcacggctacgacgtggcgatcgcgctggagtcataagcatgagtaaacaacgagtttttattgctggtcatcgcgggatggtcggttccgccatcaggcggcagctcgaacagcgcggtgatgtggaactggtattacgcacccgcgacgagctgaacctgctggacagccgcgccgtgcatgatttctttgccagcgaacgtattgaccaggtctatctggcggcggcgaaagtgggcggcattgttgccaacaacacctatccggcggatttcatctaccagaacatgatgattgagagcaacatcattcacgccgcgcatcagaacgacgtgaacaaactgctgtttctcggatcgtcctgcatctacccgaaactggcaaaacagccgatggcagaaagcgagttgttgcagggcacgctggagccgactaacgagccttatgctattgccaaaatcgccgggatcaaactgtgcgaatcatacaaccgccagtacggacgcgattaccgctcagtcatgccgaccaacctgtacgggccacacgacaacttccacccgagtaattcgcatgtgatcccagcattgctgcgtcgcttccacgaggcgacggcacagaatgcgccggacgtggtggtatggggcagcggtacaccgatgcgcgaatttctgcacgtcgatgatatggcggcggcgagcattcatgtcatggagctggcgcatgaagtctggctggagaacacccagccgatgttgtcgcacattaacgtcggcacgggcgttgactgcactatccgcgagctggcgcaaaccatcgccaaagtggtgggttacaaaggccgggtggtttttgatgccagcaaaccggatggcacgccgcgcaaactgctggatgtgacgcgcctgcatcagcttggctggtatcacgaaatctcactggaagcggggcttgccagcacttaccagtggttccttgagaatcaagaccgctttcggggggggagctaacgcgccatttaaatcaacctcagcggtcatagctgtttcctgtgactgagcaataactagcataaccccttggggcctctaaacgggtcttgaggggttttttgctgaaaccaatttgcctggcggcagtagcgcggtggtcccacctgaccccatgccgaactcagaagtgaaacgccgtagcgccgatggtagtgtggggtctccccatgcgagagtagggaactgccaggcatcaaataaaacgaaaggctcagtcgaaagactgggcctttcgggatccaggccggcctgttaacgaattaatcttccgcggcggtatcgataagcttgatatcgaattccgaagttcctattctctagaaagtataggaacttcaggtctgaagaggagtttacgtccagccaagctagcttggctgcaggtcgtcgaaattctaccgggtaggggaggcgcttttcccaaggcagtctggagcatgcgctttagcagccccgctgggcacttggcgctacacaagtggcctctggcctcgcacacattccacatccaccggtaggcgccaaccggctccgttctttggtggccccttcgcgccaccttctactcctcccctagtcaggaagttcccccccgccccgcagctcgcgtcgtgcaggacgtgacaaatggaagtagcacgtctcactagtctcgtgcagatggacagcaccgctgagcaatggaagcgggtaggcctttggggcagcggccaatagcagctttgctccttcgctttctgggctcagaggctgggaaggggtgggtccgggggcgggctcaggggcgggctcaggggcggggcgggcgcccgaaggtcctccggaggcccggcattctgcacgcttcaaaagcgcacgtctgccgcgctgttctcctcttcctcatctccgggcctttcgacctgcagcctgttgacaattaatcatcggcatagtatatcggcatagtataatacgacaaggtgaggaactaaaccatgggtcaaagtagcgatgaagccaacgctcccgttgcagggcagtttgcgcttcccctgagtgccacctttggcttaggggatcgcgtacgcaagaaatctggtgccgcttggcagggtcaagtcgtcggttggtattgcacaaaactcactcctgaaggctatgcggtcgagtccgaatcccacccaggctcagtgcaaatttatcctgtggctgcacttgaacgtgtggcctaatgaggggatcaattctctagagctcgctgatcagaagttcctattctctagaaagtataggaacttcgatggcgcctcatccctgaagccaatagggataacagggtaat

SEQ ID NO: 5 - DNA, 4844 bp, Artificial Sequence
  cscBKAR
ctatattgctgaaggtacaggcgtttccataactatttgctcgcgttttttactcaagaagaaaatgccaaatagcaacatcaggcagacaatacccgaaattgcgaagaaaactgtctggtagcctgcgtggtcaaagagtatcccagtcggcgttgaaagcagcacaatcccaagcgaactggcaatttgaaaaccaatcagaaagatcgtcgacgacaggcgcttatcaaagtttgccacgctgtatttgaagacggatatgacacaaagtggaacctcaatggcatgtaacaacttcactaatgaaataatccaggggttaacgaacagcgcgcaggaaaggatacgcaacgccataatcacaactccgataagtaatgcattttttggccctacccgattcacaaagaaaggaataatcgccatgcacagcgcttcgagtaccacctggaatgagttgagataaccatacaggcgcgttcctacatcgtgtgattcgaataaacctgaataaaagacaggaaaaagttgttgatcaaaaatgttatagaaagaccacgtccccacaataaatatgacgaaaacccagaagtttcgatccttgaaaactgcgataaaatcctctttttttacccctcccgcatctgccgctacgcactggtgatccttatctttaaaacgcatgttgatcatcataaatacagcgccaaatagcgagaccaaccagaagttgatatggggactgatactaaaaaatatgccggcaaagaacgcgccaatagcatagccaaaagatccccaggcgcgcgctgttccatattcgaaatgaaaatttcgcgccattttttcggtgaagctatcaagcaaaccgcatcccgccagataccccaagccaaaaaatagcgcccccagaattagacctacagaaaaattgctttgcagtaacggttcataaacgtaaatcataaacggtccggtcaagaccaggatgaaactcatacaccagatgagcggtttcttcagaccgagtttatcctgaacgatgccgtagaacatcataaatagaatgctggtaaactggttgaccgaataaagtgtacctaattccgtccctgtcaaccctagatgtcctttcagccaaatagcgtataacgaccaccacagcgaccaggaaataaaaaagagaaatgagtaactggatgcaaaacgatagtacgcatttctgaatggaatattcagtgccataattacctgcctgtcgttaaaaaattcacgtcctatttagagataagagcgacttcgccgtttacttctcactattccagttcttgtcgacatggcagcgctgtcattgcccctttcgccgttactgcaagcgctccgcaacgttgagcgagatcgataattcgtcgcatttctctctcatctgtagataatcccgtagaggacagacctgtgagtaacccggcaacgaacgcatctcccgcccccgtgctatcgacacaattcacagacattccagcaaaatggtgaacttgtcctcgataacagaccaccaccccttctgcacctttagtcaccaacagcatggcgatctcatactcttttgccagggcgcatatatcctgatcgttctgtgtttttccactgataagtcgccattcttcttccgagagcttgacgacatccgccagttgtagcgcctgccgcaaacacaagcggagcaaatgctcgtcttgccatagatcttcacgaatattaggatcgaagctgacaaaacctccggcatgccggatcgccgtcatcgcagtaaatgcgctggtacgcgaaggctcggcagacaacgcaattgaacagagatgtaaccattcgccatgtcgccagcagggcaagtctgtcgtctctaaaaaaagatcggcactggggcggaccataaacgtaaatgaacgttccccttgatcgttcagatcgacaagcaccgtggatgtccggtgccattcatcttgcttcagatacgtgatatcgactccctcagttagcagcgttctttgcattaacgcaccaaaaggatcatcccccacccgacctataaacccacttgttccgcctaatctggcgattcccaccgcaacgttagctggcgcgccgccaggacaaggcagtaggcgcccgtctgattctggcaagagatctacgaccgcatcccctaaaacccatactttggctgacatttttttcccttaaattcatctgagttacgcatagtgataaacctctttttcgcaaaatcgtcatggatttactaaaacatgcatattcgatcacaaaacgtcatagttaacgttaacatttgtgatattcatcgcatttatgaaagtaagggactttatttttataaaagttaacgttaacaattcaccaaatttgcttaaccaggatgattaaaatgacgcaatctcgattgcatgcggcgcaaaacgccctagcaaaacttcatgagcaccggggtaacactttctatccccattttcacctcgcgcctcctgccgggtggatgaacgatccaaacggcctgatctggtttaacgatcgttatcacgcgttttatcaacatcatccgatgagcgaacactgggggccaatgcactggggacatgccaccagcgacgatatgatccactggcagcatgagcctattgcgctagcgccaggagacgataatgacaaagacgggtgtttttcaggtagtgctgtcgatgacaatggtgtcctctcacttatctacaccggacacgtctggctcgatggtgcaggtaatgacgatgcaattcgcgaagtacaatgtctggctaccagtcgggatggtattcatttcgagaaacagggtgtgatcctcactccaccagaaggaatcatgcacttccgcgatcctaaagtgtggcgtgaagccgacacatggtggatggtagtcggggcgaaagatccaggcaacacggggcagatcctgctttatcgcggcagttcgttgcgtgaatggaccttcgatcgcgtactggcccacgctgatgcgggtgaaagctatatgtgggaatgtccggactttttcagccttggcgatcagcattatctgatgttttccccgcagggaatgaatgccgagggatacagttaccgaaatcgctttcaaagtggcgtaatacccggaatgtggtcgccaggacgactttttgcacaatccgggcattttactgaacttgataacgggcatgacttttatgcaccacaaagctttttagcgaaggatggtcggcgtattgttatcggctggatggatatgtgggaatcgccaatgccctcaaaacgtgaaggatgggcaggctgcatgacgctggcgcgcgagctatcagagagcaatggcaaacttctacaacgcccggtacacgaagctgagtcgttacgccagcagcatcaatctgtctctccccgcacaatcagcaataaatatgttttgcaggaaaacgcgcaagcagttgagattcagttgcagtgggcgctgaagaacagtgatgccgaacattacggattacagctcggcactggaatgcggctgtatattgataaccaatctgagcgacttgttttgtggcggtattacccacacgagaatttagacggctaccgtagtattcccctcccgcagcgtgacacgctcgccctaaggatatttatcgatacatcatccgtggaagtatttattaacgacggggaagcggtgatgagtagtcgaatctatccgcagccagaagaacgggaactgtcgctttatgcctcccacggagtggctgtgctgcaacatggagcactctggctactgggttaacataatatcaggtggaacaacggatcaacagcgggcaagggatccgcgtcactcttcccccttcacgaccttcaataatatgcaatgcagcttcccgcccgataatgtcatgtggaagctgaattgtggtcagcggcggtaaaaacagatgcccgacgccaaccagattatcaaagcccattacggcgacatcctgcgggattcgtacccccttcgccagaagaacctgataagccacaaaggctgcgcgatcgttaccacatatcagaacatcaaaatctggtttgcccggtttgaagtgggcattgagtaaacttgcgagatcggtgtagtgatcatcacctgttgccatgtgaaattgtttcacctcagccagatctcgtccagcatcacgccaggcctgctcaaatccctgccgacgataccctgttgccaacgcactttccggtagccagaagcataacggttgacgatagcccgccgcgagcaaatgctgtgttgattcatattgtgcagtgtaatcatcagggatataactgggtaacgctgggtcatccgccacacagttcgccaatacaatattttcaccatacagagactcaggcagcgtgatatgtcgcagccccattgtagtatagataatgccatccggacggtgggcaagcagctgacgtgccgcgcgggcagcgtcatcttcagaaaaaatattgattaaaaaactattccagccgaactcgctggcggtttgctcaatggcaagcagaatatcaacagagaaaggagtggtagccgtgtcctgcgccagcacggcgagagtcgacggcttacgtccttgagcgcgcatcttacgggcggaaagatcaggaacataattcagggtctggattgcctgcaatacgcggtcacgcgttgcaggacgcacagattctgcattatgcatcacccgggagactgtcatcat

SEQ ID NO: 6 - DNA, 4259 bp, Artificial Sequence
  galMKTE
ttactcagcaataaactgatattccgtcaggctggaatactcttcgccaggacgcaggaagcagtccggttgcggccattcagggtggttcgggctgtccggtagaaactcgctttccagagccagcccttgccagtcggcgtaaggttcggttccccgcgacggtgtgccgccgaggaagttgccggagtagaattgcagagccggagcggtggtgtagaccttcagctgcaatttttcatctgctgaccagacatgcgccgccactttcttgccatcgcctttggcctgtaacaagaatgcgtgatcgtaacctttcactttgcgctgatcgtcgtcggcaagaaactcactggcgatgattttggcgctgcggaaatcaaaagacgttccggcgacagatttcaggccgtcgtgcggaatgccgccttcatcaaccggcagatattcgtccgccagaatctgcaacttgtgattgcgcacgtcagactgctcgccgtcaagattgaaatagacgtgattagtcatattcaccgggcaaggtttatcaactgtggcgcgataagtaatggagatacggttatcgtcggtcagacgatattgcaccgtcgcgccgagattacccgggaagccctgatcaccatcatctgaactcagggcaaacagcacctgacgatcgttctggttcacaatctgccagcgacgtttgtcgaacccttccggcccgccgtgcagctggttaacgccctgacttggcgaaagcgtcacggtttcaccgtcaaaggtataacggctattggcgatacggttggcataacgaccaatagaggcccccagaaacgcggcctgatcctgatagcattccgggctggcacagccgagcagcgcctcgcggacgctgccatcggaaagcggaatacgggcggaaagtaaagtcgcaccccagtccatcagcgtgactaccatccctgcgttgttacgcaaagttaacagtcggtacggctgaccatcgggtgccagtgcgggagtttcgttcagcactgtcctgctccttgtgatggtttacaaacgtaaaaagtctctttaatacctgtttttgcttcatattgttcagcgacagcttgctgtacggcaggcaccagctcttccgggatcagcgcgacgatacagccgccaaatccgccgccggtcatgcgtacgccacctttgtcgccaatcacagctttgacgatttctaccagagtgtcaatttgcggcacggtgatttcgaaatcatcgcgcatagaggcatgagactccgccatcaactcgcccatacgtttcaggtcgccttgctccagcgcgctggcagcttcaacggtgcgggcgttttcagtcagtatatgacgcacgcgttttgccacgatcgggtccagttcatgcgcaacagcgttgaactcttcaatggtgacatcacgcagggctggctgctggaagaaacgcgcaccggtttcgcactgttcacgacgggtgttgtattcgctgccaaccagggtacgtttgaagttactgttgatgatgacgacagccacacctttgggcatggaaactgctttggtccccagtgagcggcaatcgatcagcaaggcatgatctttcttgccgagcgcggaaattagctgatccatgatcccgcagttacagcctacaaactggttttctgcttcctgaccgttaagcgcgatttgtgcgccgtccagcggcagatgataaagctgctgcaatacggttccgaccgcgacttccagtgaagcggaagaacttaacccggcaccctgcggcacattgccgctgatcaccatgtccacgccgccgaagctgttgttacgcagttgcagatgtttcaccacgccacgaacgtagttagcccattgatagttttcatgtgcgacaatgggcgcatcgagggaaaactcgtcgagctgattttcataatcggctgccatcacgcgaactttacggtcatcgcgtggtgcacaactgatcacggtttgataatcaatcgcgcagggcagaacgaaaccgtcgttgtagtcggtgtgttcaccaatcaaattcacgcggccaggcgcctgaatggtgtgagtggcagggtagccaaatgcgttggcaaacagagattgtgttttttctttcagactcatttcttacactccggattcgcgaaaatggatatcgctgactgcgcgcaaacgctctgctgcctgttctgcggtcaggtctcgctgggtctctgccagcatttcataaccaaccataaatttacgtacggtggcggagcgcagcagaggcggataaaagtgcgcgtgcagctgccagtgttgattctcttcgccattaaatggcgcgccgtgccagcccatagagtaggggaaggagcactggaagaggttgtcataacgactggtcagctttttcaacgccagcgccagatcgctgcgctgggcgtcggtcaaatcggtgatccgtaaaacgtgggctttgggcagcagtagcgtttcgaacggccaggcagcccagtaaggcacgacggctaaccagtgttcggtttcgacaacggtacggctaccgtctgccagctcgcgctgaacataatccaccagcattggtgatttctgttcggcaaaatattctttttgcaggcggtcttcgcgctcagcttcgttaggcaggaagctatttgcccaaatctgaccgtgcggatgcgggttagagcagcccatcgccgcgcctttgttttcaaaaacctgcacccatgggtacgttttccccagttctgcggtttgctcctgccaggttttgacgatttccgtcaatgctgcaacgctgagctctggcagcgttttactgtgatccggtgaaaagcagatcacccggctggtgccgcgcgcgctctggcaacgcatcagcggatcgtgactttctggcgcatctggcgtgtcagacatcaaagccgcaaagtcattagtgaaaacgtaagtcccggtgtaatcggggtttttatcgcctgtcacccgcacattacctgcgcagaggaagcaatctggatcgtgcgcaggtaacacctgtttggctggcgtttcctgcgccccctgccaggggcgcttagcgcggtgcggtgaaaccagaatccattgcccggtgagcgggttgtagcggcgatgtggatgatcaacgggattaaattgcgtcatggtcgttccttaatcgggatatccctgtggatggcgtgactgccagtgccaggtgtcctgcgccatttcatcgagtgtgcgcgttacgcgccagttcagttcacggtcggctttgctggcgtccgcccagtaggccggaaggtcgccctcgcgacgcggtgcaaaatgataattaaccggtttgccgcaggctttgctgaaggcattaaccacgtccagcacgctgttgcctacgccagcgccgaggttgtagatgtgtacgcctggcttgttcgccagtttttccatcgccacgacgtgaccgtccgccagatccattacgtggatgtaatcgcgtacgccagtaccatcttcggtcggataatcgttaccaaaaatcgccagcgagtcgcgacggcctacagcaacctgggcgatgtatggcatcaggttattcggaatgccttgcggatcttcgcccatatcgcccgacggatgcgcgccaaccgggttgaagtagcgcagcagggcaatgctccagtccggctgggctttttgcagatcggtgaggatctgttccaccatcagcttgcttttgccgtaagggctttgcggtgtgccggtcgggaagctttcaacgtatggaattttgggctgatcgccataaacggtggcggaggagctaaaaataaagtttttgacgttagcggcgcgcatggcgctaatcaggcgcagagtgccgttgacattgttgtcgtaatattccagcggtttttgtaccgattcgcccacggctttcagcccggcgaagtggatcacggtgtcgatagcgtgatcgtgcaggatctcggtcatcaacgcttcgttacgaatatcgccttcaacaaacgttggatgtttgccgcctaaacgctcgataacaggcagtacgctgcgcttactgttacagaggttatcaagaatgatgacatcatgaccgttttgcagtaattgcacacaggtatgacttccaatgtaaccgctaccaccggtaaccagaactctcat

SEQ ID NO: 7 - DNA, 4692 bp, Artificial Sequence
  pCDF-galE
ggggaattgtgagcggataacaattcccctgtagaaataattttgtttaactttaataaggagatataccaagcttgcggccgcataatgcttaagtcgaacagaaagtaatcgtattgtacacggccgcataatcgaaattaatacgactcactataggggaattgtgagcggataacaattccccatcttagtatattagttaagtataagaaggagatatacagatcacatatgagagttctggttaccggtggtagcggttacattggaagtcatacctgtgtgcaattactgcaaaacggtcatgatgtcatcattcttgataacctctgtaacagtaagcgcagcgtactgcctgttatcgagcgtttaggcggcaaacatccaacgtttgttgaaggcgatattcgtaacgaagcgttgatgaccgagatcctgcacgatcacgctatcgacaccgtgatccacttcgccgggctgaaagccgtgggcgaatcggtacaaaaaccgctggaatattacgacaacaatgtcaacggcactctgcgcctgattagcgccatgcgcgccgctaacgtcaaaaactttatttttagctcctccgccaccgtttatggcgatcagcccaaaattccatacgttgaaagcttcccgaccggcacaccgcaaagcccttacggcaaaagcaagctgatggtggaacagatcctcaccgatctgcaaaaagcccagccggactggagcattgccctgctgcgctacttcaacccggttggcgcgcatccgtcgggcgatatgggcgaagatccgcaaggcattccgaataacctgatgccatacatcgcccaggttgctgtaggccgtcgcgactcgctggcgatttttggtaacgattatccgaccgaagatggtactggcgtacgcgattacatccacgtaatggatctggcggacggtcacgtcgtggcgatggaaaaactggcgaacaagccaggcgtacacatctacaacctcggcgctggcgtaggcaacagcgtgctggacgtggttaatgccttcagcaaagcctgcggcaaaccggttaattatcattttgcaccgcgtcgcgagggcgaccttccggcctactgggcggacgccagcaaagccgaccgtgaactgaactggcgcgtaacgcgcacactcgatgaaatggcgcaggacacctggcactggcagtcacgccatccacagggatatcccgattaatgactcgagtgatctcgagtctggtaaagaaaccgctgctgcgaaatttgaacgccagcacatggactcgtctactagcgcagcttaattaacctaggctgctgccaccgctgagcaataactagcataaccccttggggcctctaaacgggtcttgaggggttttttgctgaaacctcaggcatttgagaagcacacggtcacactgcttccggtagtcaataaaccggtaaaccagcaatagacataagcggctatttaacgaccctgccctgaaccgacgaccgggtcatcgtggccggatcttgcggcccctcggcttgaacgaattgttagacattatttgccgactaccttggtgatctcgcctttcacgtagtggacaaattcttccaactgatctgcgcgcgaggccaagcgatcttcttcttgtccaagataagcctgtctagcttcaagtatgacgggctgatactgggccggcaggcgctccattgcccagtcggcagcgacatccttcggcgcgattttgccggttactgcgctgtaccaaatgcgggacaacgtaagcactacatttcgctcatcgccagcccagtcgggcggcgagttccatagcgttaaggtttcatttagcgcctcaaatagatcctgttcaggaaccggatcaaagagttcctccgccgctggacctaccaaggcaacgctatgttctcttgcttttgtcagcaagatagccagatcaatgtcgatcgtggctggctcgaagatacctgcaagaatgtcattgcgctgccattctccaaattgcagttcgcgcttagctggataacgccacggaatgatgtcgtcgtgcacaacaatggtgacttctacagcgcggagaatctcgctctctccaggggaagccgaagtttccaaaaggtcgttgatcaaagctcgccgcgttgtttcatcaagccttacggtcaccgtaaccagcaaatcaatatcactgtgtggcttcaggccgccatccactgcggagccgtacaaatgtacggccagcaacgtcggttcgagatggcgctcgatgacgccaactacctctgatagttgagtcgatacttcggcgatcaccgcttccctcatactcttcctttttcaatattattgaagcatttatcagggttattgtctcatgagcggatacatatttgaatgtatttagaaaaataaacaaatagctagctcactcggtcgctacgctccgggcgtgagactgcggcgggcgctgcggacacatacaaagttacccacagattccgtggataagcaggggactaacatgtgaggcaaaacagcagggccgcgccggtggcgtttttccataggctccgccctcctgccagagttcacataaacagacgcttttccggtgcatctgtgggagccgtgaggctcaaccatgaatctgacagtacgggcgaaacccgacaggacttaaagatccccaccgtttccggcgggtcgctccctcttgcgctctcctgttccgaccctgccgtttaccggatacctgttccgcctttctcccttacgggaagtgtggcgctttctcatagctcacacactggtatctcggctcggtgtaggtcgttcgctccaagctgggctgtaagcaagaactccccgttcagcccgactgctgcgccttatccggtaactgttcacttgagtccaacccggaaaagcacggtaaaacgccactggcagcagccattggtaactgggagttcgcagaggatttgtttagctaaacacgcggttgctcttgaagtgtgcgccaaagtccggctacactggaaggacagatttggttgctgtgctctgcgaaagccagttaccacggttaagcagttccccaactgacttaaccttcgatcaaaccacctccccaggtggttttttcgtttacagggcaaaagattacgcgcagaaaaaaaggatctcaagaagatcctttgatcttttctactgaaccgctctagatttcagtgcaatttatctcttcaaatgtagcacctgaagtcagccccatacgatataagttgtaattctcatgttagtcatgccccgcgcccaccggaaggagctgactgggttgaaggctctcaagggcatcggtcgagatcccggtgcctaatgagtgagctaacttacattaattgcgttgcgctcactgcccgctttccagtcgggaaacctgtcgtgccagctgcattaatgaatcggccaacgcgcggggagaggcggtttgcgtattgggcgccagggtggtttttcttttcaccagtgagacgggcaacagctgattgcccttcaccgcctggccctgagagagttgcagcaagcggtccacgctggtttgccccagcaggcgaaaatcctgtttgatggtggttaacggcgggatataacatgagctgtcttcggtatcgtcgtatcccactaccgagatgtccgcaccaacgcgcagcccggactcggtaatggcgcgcattgcgcccagcgccatctgatcgttggcaaccagcatcgcagtgggaacgatgccctcattcagcatttgcatggtttgttgaaaaccggacatggcactccagtcgccttcccgttccgctatcggctgaatttgattgcgagtgagatatttatgccagccagccagacgcagacgcgccgagacagaacttaatgggcccgctaacagcgcgatttgctggtgacccaatgcgaccagatgctccacgcccagtcgcgtaccgtcttcatgggagaaaataatactgttgatgggtgtctggtcagagacatcaagaaataacgccggaacattagtgcaggcagcttccacagcaatggcatcctggtcatccagcggatagttaatgatcagcccactgacgcgttgcgcgagaagattgtgcaccgccgctttacaggcttcgacgccgcttcgttctaccatcgacaccaccacgctggcacccagttgatcggcgcgagatttaatcgccgcgacaatttgcgacggcgcgtgcagggccagactggaggtggcaacgccaatcagcaacgactgtttgcccgccagttgttgtgccacgcggttgggaatgtaattcagctccgccatcgccgcttccactttttcccgcgttttcgcagaaacgtggctggcctggttcaccacgcgggaaacggtctgataagagacaccggcatactctgcgacatcgtataacgttactggtttcacattcaccaccctgaattgactctcttccgggcgctatcatgccataccgcgaaaggttttgcgccattcgatggtgtccgggatctcgacgctctcccttatgcgactcctgcattaggaaattaatacgactcactata

SEQ ID NO: 8 - DNA, 5493 bp, Artificial Sequence
  pDEST-lgtB
ttgtacaaagtggtgatgatccggctgctaacaaagcccgaaaggaagctgagttggctgctgccaccgctgagcaataactagcataaccccttggggcctctaaacgggtcttgaggggttttttgctgaaaggaggaactatatccggatatccacaggacgggtgtggtcgccatgatcgcgtagtcgatagtggctccaagtagcgaagcgagcaggactgggcggcggccaaagcggtcggacagtgctccgagaacgggtgcgcatagaaattgcatcaacgcatatagcgctagcagcacgccatagtgactggcgatgctgtcggaatggacgatatcccgcaagaggcccggcagtaccggcataaccaagcctatgcctacagcatccagggtgacggtgccgaggatgacgatgagcgcattgttagatttcatacacggtgcctgactgcgttagcaatttaactgtgataaactaccgcattaaagcttatcgatgataagctgtcaaacatgagaattcttgaagacgaaagggcctcgtgatacgcctatttttataggttaatgtcatgataataatggtttcttagacgtcaggtggcacttttcggggaaatgtgcgcggaacccctatttgtttatttttctaaatacattcaaatatgtatccgctcatgagacaataaccctgataaatgcttcaataatattgaaaaaggaagagtatgagtattcaacatttccgtgtcgcccttattcccttttttgcggcattttgccttcctgtttttgctcacccagaaacgctggtgaaagtaaaagatgctgaagatcagttgggtgcacgagtgggttacatcgaactggatctcaacagcggtaagatccttgagagttttcgccccgaagaacgttttccaatgatgagcacttttaaagttctgctatgtggcgcggtattatcccgtgttgacgccgggcaagagcaactcggtcgccgcatacactattctcagaatgacttggttgagtactcaccagtcacagaaaagcatcttacggatggcatgacagtaagagaattatgcagtgctgccataaccatgagtgataacactgcggccaacttacttctgacaacgatcggaggaccgaaggagctaaccgcttttttgcacaacatgggggatcatgtaactcgccttgatcgttgggaaccggagctgaatgaagccataccaaacgacgagcgtgacaccacgatgcctgcagcaatggcaacaacgttgcgcaaactattaactggcgaactacttactctagcttcccggcaacaattaatagactggatggaggcggataaagttgcaggaccacttctgcgctcggcccttccggctggctggtttattgctgataaatctggagccggtgagcgtgggtctcgcggtatcattgcagcactggggccagatggtaagccctcccgtatcgtagttatctacacgacggggagtcaggcaactatggatgaacgaaatagacagatcgctgagataggtgcctcactgattaagcattggtaactgtcagaccaagtttactcatatatactttagattgatttaaaacttcatttttaatttaaaaggatctaggtgaagatcctttttgataatctcatgaccaaaatcccttaacgtgagttttcgttccactgagcgtcagaccccgtagaaaagatcaaaggatcttcttgagatcctttttttctgcgcgtaatctgctgcttgcaaacaaaaaaaccaccgctaccagcggtggtttgtttgccggatcaagagctaccaactctttttccgaaggtaactggcttcagcagagcgcagataccaaatactgtccttctagtgtagccgtagttaggccaccacttcaagaactctgtagcaccgcctacatacctcgctctgctaatcctgttaccagtggctgctgccagtggcgataagtcgtgtcttaccgggttggactcaagacgatagttaccggataaggcgcagcggtcgggctgaacggggggttcgtgcacacagcccagcttggagcgaacgacctacaccgaactgagatacctacagcgtgagctatgagaaagcgccacgcttcccgaagggagaaaggcggacaggtatccggtaagcggcagggtcggaacaggagagcgcacgagggagcttccagggggaaacgcctggtatctttatagtcctgtcgggtttcgccacctctgacttgagcgtcgatttttgtgatgctcgtcaggggggcggagcctatggaaaaacgccagcaacgcggcctttttacggttcctggccttttgctggccttttgctcacatgttctttcctgcgttatcccctgattctgtggataaccgtattaccgcctttgagtgagctgataccgctcgccgcagccgaacgaccgagcgcagcgagtcagtgagcgaggaagcggaagagcgcctgatgcggtattttctccttacgcatctgtgcggtatttcacaccgcatatatggtgcactctcagtacaatctgctctgatgccgcatagttaagccagtatacactccgctatcgctacgtgactgggtcatggctgcgccccgacacccgccaacacccgctgacgcgccctgacgggcttgtctgctcccggcatccgcttacagacaagctgtgaccgtctccgggagctgcatgtgtcagaggttttcaccgtcatcaccgaaacgcgcgaggcagctgcggtaaagctcatcagcgtggtcgtgaagcgattcacagatgtctgcctgttcatccgcgtccagctcgttgagtttctccagaagcgttaatgtctggcttctgataaagcgggccatgttaagggcggttttttcctgtttggtcactgatgcctccgtgtaagggggatttctgttcatgggggtaatgataccgatgaaacgagagaggatgctcacgatacgggttactgatgatgaacatgcccggttactggaacgttgtgagggtaaacaactggcggtatggatgcggcgggaccagagaaaaatcactcagggtcaatgccagcgcttcgttaatacagatgtaggtgttccacagggtagccagcagcatcctgcgatgcagatccggaacataatggtgcagggcgctgacttccgcgtttccagactttacgaaacacggaaaccgaagaccattcatgttgttgctcaggtcgcagacgttttgcagcagcagtcgcttcacgttcgctcgcgtatcggtgattcattctgctaaccagtaaggcaaccccgccagcctagccgggtcctcaacgacaggagcacgatcatgcgcacccgtggccaggacccaacgctgcccgagatgcgccgcgtgcggctgctggagatggcggacgcgatggatatgttctgccaagggttggtttgcgcattcacagttctccgcaagaattgattggctccaattcttggagtggtgaatccgttagcgaggtgccgccggcttccattcaggtcgaggtggcccggctccatgcaccgcgacgcaacgcggggaggcagacaaggtatagggcggcgcctacaatccatgccaacccgttccatgtgctcgccgaggcggcataaatcgccgtgacgatcagcggtccagtgatcgaagttaggctggtaagagccgcgagcgatccttgaagctgtccctgatggtcgtcatctacctgcctggacagcatggcctgcaacgcgggcatcccgatgccgccggaagcgagaagaatcataatggggaaggccatccagcctcgcgtcgcgaacgccagcaagacgtagcccagcgcgtcggccgccatgccggcgataatggcctgcttctcgccgaaacgtttggtggcgggaccagtgacgaaggcttgagcgagggcgtgcaagattccgaataccgcaagcgacaggccgatcatcgtcgcgctccagcgaaagcggtcctcgccgaaaatgacccagagcgctgccggcacctgtcctacgagttgcatgataaagaagacagtcataagtgcggcgacgatagtcatgccccgcgcccaccggaaggagctgactgggttgaaggctctcaagggcatcggtcgatcgacgctctcccttatgcgactcctgcattaggaagcagcccagtagtaggttgaggccgttgagcaccgccgccgcaaggaatggtgcatgcaaggagatggcgcccaacagtcccccggccacggggcctgccaccatacccacgccgaaacaagcgctcatgagcccgaagtggcgagcccgatcttccccatcggtgatgtcggcgatataggcgccagcaaccgcacctgtggcgccggtgatgccggccacgatgcgtccggcgtagaggatcgagatctcgatcccgcgaaattaatacgactcactatagggagaccacaacggtttccctctagatcacaagtttgtacaaaaaagcaggcttcgaaggagatagaaccatggcccaccatcaccatcaccatcaaaaccacgttatcagcttagcttccgccgcagaacgcagggcgcacattgccgataccttcggcaggcacggcatcccgtttcagtttttcgacgcactgatgccgtctgaaaggctggaacaggcaatggcggaactcgtccccggcttgtcggcgcacccctatttgagcggagtggaaaaagcctgctttatgagccacgccgtattgtggaagcaggcattggacgaaggtctgccgtatatcaccgtatttgaggacgacgttttactcggcgaaggtgcggaaaaattccttgccgaagacgcttggctgcaagaacgctttgacccggataccgcctttatcgtccgcttggaaacgatgtttatgcacgtcctgacctcgccctccggcgtggcggattactgcgggcgcgcctttccgctgttggaaagcgaacactgggggacggcgggctatatcatttcccgaaaagcgatgcggtttttcctggacaggtttgccgccctgccgcccgaagggctgcaccccgtcgatctgatgatgttcagcgattttttcgacagggaaggaatgccggtttgccagctcaatcccgccttgtgcgcccaagagctgcattatgccaagtttcacgaccaaaacagcgcattgggcagcctgatcgaacacgaccgcctcctgaaccgcaaacagcaaaggcgcgattcccccgccaacacattcaaacaccgcctgatccgcgccttgaccgatatcagcagggaaagggaaaaacgccggcaaaggcgcgaacagttcattgtgcctttccaataagacccagctttc

SEQ ID NO: 9 - DNA, 4568 bp, Artificial Sequence
  Ptet-lgtA-PT5-galT-FRT-kanR-FRT
acaggttggctgataagtccccggtctagcttgcatgcagattgcagcattacacgtcttgagcgattgtgtaggctggagctgcttcgaagttcctatactttctagagaataggaacttcggaataggaacttcatttaaatggcgcgccttacgccccgccctgccggtaccgagagcgcttttgaagctggggtgggcgaagaactccagcatgagatccccgcgctggaggatcatccagccggcgtcccggaaaacgattccgaagcccaacctttcatagaaggcggcggtggaatcgaaatctcgtgatggcaggttgggcgtcgcttggtcggtcatttcgaaccccagagtcccgctcagaagaactcgtcaagaaggcgatagaaggcgatgcgctgcgaatcgggagcggcgataccgtaaagcacgaggaagcggtcagcccattcgccgccaagctcttcagcaatatcacgggtagccaacgctatgtcctgatagcggtccgccacacccagccggccacagtcgatgaatccagaaaagcggccattttccaccatgatattcggcaagcaggcatcgccatgggtcacgacgagatcctcgccgtcgggcatgcgcgccttgagcctggcgaacagttcggctggcgcgagcccctgatgctcttcgtccagatcatcctgatcgacaagaccggcttccatccgagtacgtgctcgctcgatgcgatgtttcgcttggtggtcgaatgggcaggtagccggatcaagcgtatgcagccgccgcattgcatcagccatgatggatactttctcggcaggagcaaggtgagatgacaggagatcctgccccggcacttcgcccaatagcagccagtcccttcccgcttcagtgacaacgtcgagcacagctgcgcaaggaacgcccgtcgtggccagccacgatagccgcgctgcctcgtcctgcagttcattcagggcaccggacaggtcggtcttgacaaaaagaaccgggcgcccctgcgctgacagccggaacacggcggcatcagagcagccgattgtctgttgtgcccagtcatagccgaatagcctctccacccaagcggccggagaacctgcgtgcaatccatcttgttcaatcatgcgaaacgatcctcatcctgtctcttgatcagatcttgatcccctgcgccatcagatccttggcggcaagaaagccatccagtttactttgcagggcttcccaaccttaccagagggcgccccagctggcaattccggttcgcttgctgtccataaaaccgcccagtctagctatcgccatgtaagcccactgcaagctacctgctttctctttgcgcttgcgttttcccttgtccagatagcccagtagctgacattcatccggggtcagcaccgtttctgcggactggctttctacgtgttccgcttcctttagcagcccttgcgccctgagtgcttgcggcagcgtgaggggatcttgacgcgtgtcacaggtaggacgcgccgaagttcctatactttctagagaataggaacttcggaataggaactaaggaggatattcatacatgatggtagtgttcgaaattaatacgactcactataggggaattgattctggtaccaaatgagtcgaccggccagatgattaattcctaatttttgttgacactctatcattgatagagttattttaccactccctatcagtgatagagaaaagtgaaatgaatagttcgacaaaaatctagaaataattttgtttaactttaagaaggagatatacaaatgccgtccgaagcattccgtcgtcaccgtgcttatcgcgaaaacaaactgcagccactggtctctgtcctgatctgcgcatacaacgttgagaaatacttcgcacagtctctggcagctgtagttaaccagacctggcgtaacctggatatcctgatcgtagatgacggctctacggatggtacgctggcgatcgcacagcgtttccaggaacaggacggtcgtatccgcattctcgctcagccgcgtaactctggtctgatcccgtctctgaacatcggtctggacgaactggccaaatctggtggtggtggcgaatacatcgcccgtactgacgccgacgacattgcggccccggattggatcgaaaaaatcgtaggtgaaatggagaaagaccgctctatcatcgcgatgggtgcttggctggaagttctgtccgaagagaaagacggtaaccgtctggcccgtcaccatgaacacggcaaaatctggaaaaaaccgacccgtcacgaagatatcgcggacttcttcccgttcggtaacccgatccataacaacaccatgatcatgcgtcgtagcgtaatcgacggtggtctgcgttacaacaccgaacgtgattgggcagaagactaccagttttggtatgacgtgtctaaactgggtcgtctggcttactacccagaagcgctggttaaataccgtctgcacgccaaccaggttagctccaaatactccatccgtcagcacgaaatcgcacagggtatccagaaaacggctcgtaacgacttcctgcagtccatgggtttcaaaacccgtttcgactctctggagtaccgtcagatcaaagcggttgcgtatgagctgctggagaaacacctgccggaagaggactttgaacgtgcgcgtcgtttcctgtaccagtgcttcaaacgtaccgacactctgccggcgggtgcatggctcgactttgcagcggatggtcgtatgcgtcgtctgtttaccctgcgtcagtacttcggtatcctgcatcgtctcctgaaaaaccgctaatgatttcgtcgacacacaggaaacatattaaaaattaaaacctgcaggagtttaaacgcggccgcgatatcgttgtaaaacgacggccagtgcaagaatcataaaaaatttatttgctttcaggaaaatttttctgtataatagattcataaatttgagagaggagtttttgtgagcggataacaattccccatcttagtatattagttaagtataaatacacaaggagatataccatgacgcaatttaatcccgttgatcatccacatcgccgctacaacccgctcaccgggcaatggattctggtttcaccgcaccgcgctaagcgcccctggcagggggcgcaggaaacgccagccaaacaggtgttacctgcgcacgatccagattgcttcctctgcgcaggtaatgtgcgggtgacaggcgataaaaaccccgattacaccgggacttacgttttcactaatgactttgcggctttgatgtctgacacgccagatgcgccagaaagtcacgatccgctgatgcgttgccagagcgcgcgcggcaccagccgggtgatctgcttttcaccggatcacagtaaaacgctgccagagctcagcgttgcagcattgacggaaatcgtcaaaacctggcaggagcaaaccgcagaactggggaaaacgtacccatgggtgcaggtttttgaaaacaaaggcgcggcgatgggctgctctaacccgcatccgcacggtcagatttgggcaaatagcttcctgcctaacgaagctgagcgcgaagaccgcctgcaaaaagaatattttgccgaacagaaatcaccaatgctggtggattatgttcagcgcgagctggcagacggtagccgtaccgttgtcgaaaccgaacactggttagccgtcgtgccttactgggctgcctggccgttcgaaacgctactgctgcccaaagcccacgttttacggatcaccgatttgaccgacgcccagcgcagcgatctggcgctggcgttgaaaaagctgaccagtcgttatgacaacctcttccagtgctccttcccctactctatgggctggcacggcgcgccatttaatggcgaagagaatcaacactggcagctgcacgcgcacttttatccgcctctgctgcgctccgccaccgtacgtaaatttatggttggttatgaaatgctggcagagacccagcgagacctgaccgcagaacaggcagcagagcgtttgcgcgcagtcagcgatatccattttcgcgaatccggagtgtaacgcggaggcgcgccatttaaatcaacctcagcggtcatagctgtttcctgtgactgagcaataactagcataaccccttggggcctctaaacgggtcttgaggggttttttgctgaaaccaatttgcctggcggcagtagcgcggtggtcccacctgaccccatgccgaactcagaagtgaaacgccgtagcgccgatggtagtgtggggtctccccatgcgagagtagggaactgccaggcatcaaataaaacgaaaggctcagtcgaaagactgggcctttcgggatccaggccggcctgttaacgaattaatcttccgcggcaacaaaaattaggaattaatcatctggccaatttcaggtggcacttttcgggcagaccggggacttatcagccaacctgt

SEQ ID NO: 10 - DNA, 6521 bp, Artificial Sequence
  Ptet-glmUM-PT5-glmS-FRT-dhfr-FRT
acaggttggctgataagtccccggtctagcttgcatgcagattgcagcattacacgtcttgagcgattgtgtaggctggagctgcttcgaaattaatacgactcactataggggaattgattctggtaccaaatgagtcgaccggccagatgattaattcctaatttttgttgacactctatcattgatagagttattttaccactccctatcagtgatagagaaaagtgaaatgaatagttcgacaaaaatctagaaataattttgtttaactttaagaaggagatatacaaatgctgaacaacgcgatgtctgttgttatcctggcggcgggtaaaggtacccgtatgtactctgacctgccgaaagttctgcacaccctggcgggtaaagcgatggttcagcacgttatcgacgcggcgaacgaactgggtgcggcgcacgttcacctggtttacggtcacggtggtgacctgctgaaacaggcgctgaaagacgacaacctgaactgggttctgcaggcggaacagctgggtaccggtcacgcgatgcagcaggcggcgccgttcttcgcggacgacgaagacatcctgatgctgtacggtgacgttccgctgatctctgttgaaaccctgcagcgtctgcgtgacgcgaaaccgcagggtggtatcggtctgctgaccgttaaactggacgacccgaccggttacggtcgtatcacccgtgaaaacggtaaagtaaccggtatcgttgaacacaaagacgcgaccgacgaacagcgtcagatccaggagatcaacaccggtatcctgatcgcgaacggtgcagacatgaaacgttggctggcgaaactgaccaacaacaacgcgcagggtgaatactacatcaccgacatcatcgcgctggcgtaccaggaaggtcgtgaaatcgttgcggttcacccgcagcgtctgtctgaagttgaaggtgttaacaaccgtctgcagctgtctcgtctggaacgtgtttaccagtctgaacaggcggaaaaactgctgctggcgggtgttatgctgcgtgacccggcgcgtttcgacctgcgtggtaccctgacccacggtcgtgacgttgaaatcgacaccaacgttatcatcgaaggtaacgttaccctgggtcaccgtgtaaaaatcggcaccggttgcgttatcaaaaactctgttatcggtgacgactgcgaaatctctccgtacaccgttgttgaagacgcgaacctggcggcggcgtgcaccatcggtccgttcgcgcgtctgcgtccgggtgcggaactgctggaaggtgcgcacgttggtaacttcgttgaaatgaaaaaagcgcgtctgggtaaaggttctaaagcgggtcacctgacctacctgggtgacgcggaaatcggtgacaacgttaacatcggtgcgggtaccatcacctgcaactacgacggtgcgaacaaattcaaaaccatcatcggtgacgacgttttcgttggttctgacacccagctggttgcgccggttaccgttggtaaaggtgcgaccatcgcggcgggtaccaccgttacccgtaacgttggtgaaaacgcgctggcgatctctcgtgttccgcagacccagaaagaaggttggcgtcgtccggttaaaaaaaaataacgaaggagatagaaccatgtccaaccgtaaatacttcggtacggacggtatccgtggtcgtgtaggtgatgctccgattacgccggatttcgtcctgaaactcggttgggcagcgggtaaagttctcgcacgtcacggctctcgtaaaatcatcatcggtaaagacacccgtatctctggttacatgctcgaatctgcactggaagcgggtctggctgcagctggtctgtctgcactgttcacgggtccgatgccaaccccagctgtagcgtacctgactcgcactttccgtgcagaagcaggtatcgtgatctctgcctctcacaacccgttctacgacaacggtatcaaattcttcagcatcgatggtaccaaactcccagacgcggttgaagaggctatcgaagcggaaatggagaaagaaatctcttgtgtagactctgccgaactcggtaaagcgtctcgtatcgttgatgcagcgggtcgttacatcgagttctgcaaagccacctttccgaacgaactgagcctgtctgagctgaaaatcgtcgtagactgtgccaacggtgcgacttaccacattgccccaaacgtactgcgtgagctgggtgctaacgtcatcgcgatcggttgtgaaccgaacggtgtcaacatcaacgcggaagtaggtgcgaccgatgttcgtgcactgcaggctcgtgtactcgcggagaaagcggatctcggtatcgcctttgacggtgatggtgaccgtgttatcatggttgaccacgaaggtaacaaagtggatggtgaccagatcatgtacatcattgcccgtgaaggtctgcgtcagggtcagctgcgtggtggtgcagtaggtaccctcatgagcaacatgggtctggaactggccctgaaacagctgggtatcccattcgctcgtgctaaagtaggcgaccgttacgttctggagaaaatgcaggagaaaggttggcgtatcggtgccgaaaactctggtcacgtcatcctgctggacaaaaccactaccggtgacggtatcgtagcaggtctgcaggtactcgccgctatggcccgtaaccacatgtccctccatgacctctgctctggtatgaaaatgttcccgcagatcctggttaacgttcgttacaccgcaggttctggtgatccgctggaacacgagtctgtgaaagccgttaccgcagaagtggaagcggccctgggtaaccgtggtcgtgtactgctgcgtaaatccggtactgagccactgatccgtgttatggttgagggcgaagatgaagcccaggtcaccgaatttgcgcaccgtattgccgacgcagtcaaagcggtttaatttcgtcgacacacaggaaacatattaaaaattaaaacctgcaggagtttaaacgcggccgcgatatcgttgtaaaacgacggccagtgcaagaatcataaaaaatttatttgctttcaggaaaatttttctgtataatagattcataaatttgagagaggagtttttgtgagcggataacaattccccatcttagtatattagttaagtataaatacacaaggagatatacatatgtgcggtatcgttggtgctatcgcacagcgtgatgtagcggagatcctcctggaaggtctgcgtcgtctcgaataccgtggttacgactctgccggtctggcagtagtggatgcagaaggtcacatgactcgtctgcgtcgtctgggtaaagtgcagatgctcgcgcaggcggcggaagaacacccactccacggtggtacgggtatcgcacacactcgttgggcaacccacggtgaaccgtctgaggtcaacgcacacccgcatgttagcgagcacatcgtagtcgttcacaacggtatcatcgagaaccacgaaccactccgtgaggaactcaaagcccgtggttacaccttcgtaagcgaaaccgacacggaagttatcgcccacctcgttaactgggaactcaaacagggtggtactctgcgtgaagcagttctgcgtgccattccacagctgcgtggtgcatacggtaccgtgatcatggactctcgtcatccggataccctgctcgccgcacgttctggttctccactcgttatcggtctgggtatgggtgagaacttcatcgcctctgatcagctggccctgctcccagttacccgtcgcttcatcttcctggaagagggtgacatcgccgaaatcacccgtcgttccgttaacatcttcgacaaaacgggtgcggaagttaaacgtcaggacatcgagtctaacctgcagtatgacgctggtgacaaaggcatctaccgtcactacatgcagaaagagatctacgaacagccgaacgcgatcaaaaacaccctgaccggtcgtatctctcacggtcaggttgacctgtctgagctgggtccaaacgcggacgaactcctgtccaaagtcgagcacatccagatcctggcttgtggtacctcttacaactccggtatggtttctcgttactggttcgaatctctggcaggtatcccatgcgacgttgaaatcgcctccgaattccgttatcgtaaatctgcggtacgtcgtaactccctcatgatcaccctgtctcagtctggtgaaaccgctgatactctggcaggtctgcgtctcagcaaagaactgggttacctgggttctctggccatctgcaacgttccgggttctagcctggttcgtgagtctgacctggctctgatgaccaacgcgggtacggagatcggtgttgcctctaccaaagcgttcactacccagctcactgtcctgctgatgctggttgccaaactgtctcgtctcaaaggcctcgacgctagcatcgaacacgacatcgtacacggtctgcaggccctcccatctcgtatcgagcagatgctgtctcaggacaaacgtatcgaagcactggcagaagacttcagcgacaaacaccacgcgctgtttctgggtcgtggtgaccagtacccaattgcgctggaaggtgccctgaaactgaaagagatcagctacatccatgcagaggcatacgcagcgggtgagctgaaacatggtccactggccctgatcgacgcagatatgccggttattgtggttgctccgaacaacgaactgctggagaaactgaaatccaacatcgaggaagtacgtgcgcgtggtggtcagctgtacgtgtttgctgaccaggacgcgggtttcgtttccagcgacaacatgcacatcatcgaaatgccgcatgttgaagaggtaatcgcgccaatcttctacaccgtaccgctgcagctgctggcgtaccatgtagccctgatcaaaggtacggacgttgaccagccgcgtaacctggcgaaatccgtgaccgtggaataacgcggaggcgcgccatttaaatcaacctcagcggtcatagctgtttcctgtgactgagcaataactagcataaccccttggggcctctaaacgggtcttgaggggttttttgctgaaaccaatttgcctggcggcagtagcgcggtggtcccacctgaccccatgccgaactcagaagtgaaacgccgtagcgccgatggtagtgtggggtctccccatgcgagagtagggaactgccaggcatcaaataaaacgaaaggctcagtcgaaagactgggcctttcgggatccaggccggcctgttaacgaattaatcttccgcggcggtatcgataagcttgatatcgaattccgaagttcctattctctagaaagtataggaacttcaggtctgaagaggagtttacgtccagccaagctagcttggctgcaggtcgtcgaaattctaccgggtaggggaggcgcttttcccaaggcagtctggagcatgcgctttagcagccccgctgggcacttggcgctacacaagtggcctctggcctcgcacacattccacatccaccggtaggcgccaaccggctccgttctttggtggccccttcgcgccaccttctactcctcccctagtcaggaagttcccccccgccccgcagctcgcgtcgtgcaggacgtgacaaatggaagtagcacgtctcactagtctcgtgcagatggacagcaccgctgagcaatggaagcgggtaggcctttggggcagcggccaatagcagctttgctccttcgctttctgggctcagaggctgggaaggggtgggtccgggggcgggctcaggggcgggctcaggggcggggcgggcgcccgaaggtcctccggaggcccggcattctgcacgcttcaaaagcgcacgtctgccgcgctgttctcctcttcctcatctccgggcctttcgacctgcagcctgttgacaattaatcatcggcatagtatatcggcatagtataatacgacaaggtgaggaactaaaccatgggtcaaagtagcgatgaagccaacgctcccgttgcagggcagtttgcgcttcccctgagtgccacctttggcttaggggatcgcgtacgcaagaaatctggtgccgcttggcagggtcaagtcgtcggttggtattgcacaaaactcactcctgaaggctatgcggtcgagtccgaatcccacccaggctcagtgcaaatttatcctgtggctgcacttgaacgtgtggcctaatgaggggatcaattctctagagctcgctgatcagaagttcctattctctagaaagtataggaacttcgatggcgcctcatccctgaagccaatacaacaaaaattaggaattaatcatctggccaatttcaggtggcacttttcgggcagaccggggacttatcagccaacctgt

SEQ ID NO: 11 - DNA, 4187 bp, Artificial Sequence
  PT5-lgtB-FRT-tetR-FRT
cacaggttggctgataagtccccggtctagcttgcatgcagattgcagcattacacgtcttgagcgattgtgtaggctggagctgctcaagcccgtcagggcgcgtcagcgggtgttggcgggtgtcggggctggcttaactatgcggcatcagagcagattgtactgagagtgcaccatatgcggtgtgaaataccgcacagatgcgtaaggagaaaataccgcatcaggcgccattcgccattcaggctgcgcaactgttgggaagggcgatcggtgcgggcctcttcgctattacgccagctggcgaaagggggatgtgctgcaaggcgattaagttgggtaacgccagggttttcccagtcacgacgttgtaaaacgacggccagtgaattcgagctcggtacctcgcgaatgcatctagattgtaaaacgacggccagtgaattcccttagggataacagggtaattacggccccaaggtccaaacggtgaaggtaccgggccccccctcgaggtcgaggtacccaaatatgcataatcgaaattaatacgactcactataggggaattgattctggtaccaaatgagtcgaccggccagatgattaattcctaatttttgttgacactctatcattgatagagttattttaccactccctatcagtgatagagaaaagtgaaatgaatagttcgacaaaaatctagaaataattttgtttaactttaagaaggagatatacaatttcgtcgacacacaggaaacatattaaaaattaaaacctgcaggagtttaaacgcggccgcgatatcgttgtaaaacgacggccagtgcaagaatcataaaaaatttatttgctttcaggaaaatttttctgtataatagattcataaatttgagagaggagtttttgtgagcggataacaattccccatcttagtatattagttaagtataaatacaccgcggaggcgtcgaaggagatacaaccatgcaaaaccacgttatcagcttagcttccgccgcagaacgcagggcgcacattgccgataccttcggcaggcacggcatcccgtttcagtttttcgacgcactgatgccgtctgaaaggctggaacaggcaatggcggaactcgtccccggcttgtcggcgcacccctatttgagcggagtggaaaaagcctgctttatgagccacgccgtattgtggaagcaggcattggacgaaggtctgccgtatatcaccgtatttgaggacgacgttttactcggcgaaggtgcggaaaaattccttgccgaagacgcttggctgcaagaacgctttgacccggataccgcctttatcgtccgcttggaaacgatgtttatgcacgtcctgacctcgccctccggcgtggcggattactgcgggcgcgcctttccgctgttggaaagcgaacactgggggacggcgggctatatcatttcccgaaaagcgatgcggtttttcctggacaggtttgccgccctgccgcccgaagggctgcaccccgtcgatctgatgatgttcagcgattttttcgacagggaaggaatgccggtttgccagctcaatcccgccttgtgcgcccaagagctgcattatgccaagtttcacgaccaaaacagcgcattgggcagcctgatcgaacacgaccgcctcctgaaccgcaaacagcaaaggcgcgattcccccgccaacacattcaaacaccgcctgatccgcgccttgaccgatatcagcagggaaagggaaaaacgccggcaaaggcgcgaacagttcattgtgcctttccaataacgccatttaaatcaacctcagcggtcatagctgtttcctgtgactgagcaataactagcataaccccttggggcctctaaacgggtcttgaggggttttttgctgaaaccaatttgcctggcggcagtagcgcggtggtcccacctgaccccatgccgaactcagaagtgaaacgccgtagcgccgatggtagtgtggggtctccccatgcgagagtagggaactgccaggcatcaaataaaacgaaaggctcagtcgaaagactgggcctttcgggatccaggccggcctgttaacgaattaatcttccgcggcggtatcgataagcttgatatcgacactaccatcatgtatgaatatcctccttagttcctattccgaagttcctattctctagaaagtataggaacttcggcgacgtctaagaaaccattattatcatgacattaacctataaaaataggcgtatcacgaggccctttcgtcttcaagaattctcatgtttgacagcttatcatcgataagctttaatgcggtagtttatcacagttaaattgctaacgcagtcaggcaccgtgtatgaaatctaacaatgcgctcatcgtcatcctcggcaccgtcaccctggatgctgtaggcataggcttggttatgccggtactgccgggcctcttgcgggatatcgtccattccgacagcatcgccagtcactatggcgtgctgctagcgctatatgcgttgatgcaatttctatgcgcacccgttctcggagcactgtccgaccgctttggccgccgcccagtcctgctcgcttcgctacttggagccactatcgactacgcgatcatggcgaccacacccgtcctgtggatcctctacgccggacgcatcgtggccggcatcaccggcgccacaggtgcggttgctggcgcctatatcgccgacatcaccgatggggaagatcgggctcgccacttcgggctcatgagcgcttgtttcggcgtgggtatggtggcaggccccgtggccgggggactgttgggcgccatctccttgcatgcaccattccttgcggcggcggtgctcaacggcctcaacctactactgggctgcttcctaatgcaggagtcgcataagggagagcgtcgaccgatgcccttgagagccttcaacccagtcagctccttccggtgggcgcggggcatgactatcgtcgccgcacttatgactgtcttctttatcatgcaactcgtaggacaggtgccggcagcgctctgggtcattttcggcgaggaccgctttcgctggagcgcgacgatgatcggcctgtcgcttgcggtattcggaatcttgcacgccctcgctcaagccttcgtcactggtcccgccaccaaacgtttcggcgagaagcaggccattatcgccggcatggcggccgacgcgctgggctacgtcttgctggcgttcgcgacgcgaggctggatggccttccccattatgattcttctcgcttccggcggcatcgggatgcccgcgttgcaggccatgctgtccaggcaggtagatgacgaccatcagggacagcttcaaggatcgctcgcggctcttaccagcctaacttcgatcattggaccgctgatcgtcacggcgatttatgccgcctcggcgagcacatggaacgggttggcatggattgtaggcgccgccctataccttgtctgcctccccgcgttgcgtcgcggtgcatggagccgggccacctcgacctgagtggcagggcggggcgtaaggcgcgccatttaaatgaagttcctattccgaagttcctattctctagaaagtataggaacttcgaagcagctccagcctacacaatcgctcaagacgtgtaatgctgcaatctgcatgcaagcttggcactgggatggcgcctcatccctgaagccaatagggataacagggtaataagcttggcgtaatcatgtcatgatcggatcccgggcccgtcgactgcagaggcctgcatgcaagcttggcgtaatcatggtcatagctgtttcctgtgtgaaattgttatccgctcacaattccacacaacatacgagccggaagcataaagtgtaaagcctggggtgcctaatgagtgagctaactcacattaattgcgttgcgctcactgcccgctttccagtcgggaaacctgtcgtgccagctgcattaatgaatcggccaacgcgcggggagaggcggtttgcgtattgggcgctcttccgcttcctcgccaacaaaaattaggaattaatcatctggccaatttcaggtggcacttttcgggcagaccggggacttatcagccaacctgt

SEQ ID NO: 12 - DNA, 2836 bp, Artificial Sequence
  Pt5-galE-FRT-cat-FRT
agtttaaacgcggccgcgatatcgttgtaaaacgacggccagtgcaagaatcataaaaaatttatttgctttcaggaaaatttttctgtataatagattcataaatttgagagaggagtttttgtgagcggataacaattccccatcttagtatattagttaagtataaatacaccgcggaggcgtcgaaggagatacaaccatgagagttctggttaccggtggtagcggttacattggaagtcatacctgtgtgcaattactgcaaaacggtcatgatgtcatcattcttgataacctctgtaacagtaagcgcagcgtactgcctgttatcgagcgtttaggcggcaaacatccaacgtttgttgaaggcgatattcgtaacgaagcgttgatgaccgagatcctgcacgatcacgctatcgacaccgtgatccacttcgccgggctgaaagccgtgggcgaatcggtacaaaaaccgctggaatattacgacaacaatgtcaacggcactctgcgcctgattagcgccatgcgcgccgctaacgtcaaaaactttatttttagctcctccgccaccgtttatggcgatcagcccaaaattccatacgttgaaagcttcccgaccggcacaccgcaaagcccttacggcaaaagcaagctgatggtggaacagatcctcaccgatctgcaaaaagcccagccggactggagcattgccctgctgcgctacttcaacccggttggcgcgcatccgtcgggcgatatgggcgaagatccgcaaggcattccgaataacctgatgccatacatcgcccaggttgctgtaggccgtcgcgactcgctggcgatttttggtaacgattatccgaccgaagatggtactggcgtacgcgattacatccacgtaatggatctggcggacggtcacgtcgtggcgatggaaaaactggcgaacaagccaggcgtacacatctacaacctcggcgctggcgtaggcaacagcgtgctggacgtggttaatgccttcagcaaagcctgcggcaaaccggttaattatcattttgcaccgcgtcgcgagggcgaccttccggcctactgggcggacgccagcaaagccgaccgtgaactgaactggcgcgtaacgcgcacactcgatgaaatggcgcaggacacctggcactggcagtcacgccatccacagggatatcccgattaacgccatttaaatcaacctcagcggtcatagctgtttcctgtgactgagcaataactagcataaccccttggggcctctaaacgggtcttgaggggttttttgctgaaaccaatttgcctggcggcagtagcgcggtggtcccacctgaccccatgccgaactcagaagtgaaacgccgtagcgccgatggtagtgtggggtctccccatgcgagagtagggaactgccaggcatcaaataaaacgaaaggctcagtcgaaagactgggcctttcgggatccaggccggcctgttaacgaattaatcttccgcggcggtatcgataagcttgatatcgaggctgacatgggaattagccatggtccatatgaatatcctccttagttcctattccgaagttcctattctctagaaagtataggaacttcggcgcgcctacctgtgacggaagatcacttcgcagaataaataaatcctggtgtccctgttgataccgggaagccctgggccaacttttggcgaaaatgagacgttgatcggcacgtaagaggttccaactttcaccataatgaaataagatcactaccgggcgtattttttgagttgtcgagattttcaggagctaaggaagctaaaatggagaaaaaaatcactggatataccaccgttgatatatcccaatggcatcgtaaagaacattttgaggcatttcagtcagttgctcaatgtacctataaccagaccgttcagctggatattacggcctttttaaagaccgtaaagaaaaataagcacaagttttatccggcctttattcacattcttgcccgcctgatgaatgctcatccggaattacgtatggcaatgaaagacggtgagctggtgatatgggatagtgttcacccttgttacaccgttttccatgagcaaactgaaacgttttcatcgctctggagtgaataccacgacgatttccggcagtttctacacatatattcgcaagatgtggcgtgttacggtgaaaacctggcctatttccctaaagggtttattgagaatatgtttttcgtctcagccaatccctgggtgagtttcaccagttttgatttaaacgtggccaatatggacaacttcttcgcccccgttttcaccatgggcaaatattatacgcaaggcgacaaggtgctgatgccgctggcgattcaggttcatcatgccgtttgtgatggcttccatgtcggcagatgcttaatgaatacaacagtactgcgatgagtggcagggcggggcgtaaggcgcgccatttaaatgaagttcctattccgaagttcctattctctagaaagtataggaacttcgaagcagctccagcctacacaatcgctcaagacgtgtaatgctgcaatctgcatgcaagcttggcactggcgatggcgcctcatccctgaagccaatagggataacagggtaatgatcggatcccgggcccgtcgactgcagaggcctgcatgcaagcttggcgtaatcatggtcatagctgtttcctgtgtgaaattgttatccgctcacaattccacacaacatacgagccggaagcataaagtgtaaagcctgggg

SEQ ID NO: 13 - DNA, 6770 bp, Artificial Sequence
  pINT-malE-lgtB
tcgcgcgtttcggtgatgacggtgaaaacctctgacacatgcagctcccggagacggtcacagcttgtctgtaagcggatgccgggagcagacaagcccgtcagggcgcgtcagcgggtgttggcgggtgtcggggctggcttaactatgcggcatcagagcagattgtactgagagtgcaccatatgcggtgtgaaataccgcacagatgcgtaaggagaaaataccgcatcaggcgccattcgccattcaggctgcgcaactgttgggaagggcgatcggtgcgggcctcttcgctattacgccagctggcgaaagggggatgtgctgcaaggcgattaagttgggtaacgccagggttttcccagtcacgacgttgtaaaacgacggccagtgaattcgaagatcctttgatcttttctacggggtctgacgctcagtggaacgaaaactcacgttaagggattttggtcatgagattatcaaaaaggatcttcacctagatccttttaaactagtgaagttaccatcacggaaaaaggttatgctgcttttaagacccactttcacatttaagttgtttttctaatccgcatatgatcaattcaaggccgaataagaaggctggctctgcaccttggtgatcaaataattcgatagcttgtcgtaataatggcggcatactatcagtagtaggtgtttccctttcttctttagcgacttgatgctcttgatcttccaatacgcaacctaaagtaaaatgccccactgcgctgagtgcatataatgcattctctagtgaaaaaccttgttggcataaaaaggctaattgattttcgagagtttcatactgtttttctgtaggccgtgtacctaaatgtacttttgctccatcgcgatgacttagtaaagcacatctaaaacttttagcgttattacgtaaaaaatcttgccagctttccccttctaaagggcaaaagtgagtatggtgcctatctaacatctcaatggctaaggcgtcgagcaaagcccgcttattttttacatgccaatacaatgtaggctgctctacacctagcttctgggcgagtttacgggttgttaaaccttcgattccgacctcattaagcagctctaatgcgctgttaatcactttacttttatctaaacgagacatactcttcctttttcaatattattgaagcatttatcagggttattgtctcatgagcggatacatatttgaatgtatttagaaaaataaacaaataggggttccgcgcacatttccccgaaaagtgccacctgaaattggccagatgattaattcctaatttttgttgacactctatcattgatagagttattttaccactccctatcagtgatagagaaaagtgaaatgaatagttcgacaaaaatctagaaataattttgtttaactttaagaaggagatatacaaatgaaaatcgaagaaggtaaactggtaatctggattaacggcgataaaggctataacggtctcgctgaagtcggtaagaaattcgagaaagataccggaattaaagtcaccgttgagcatccggataaactggaagagaaattcccacaggttgcggcaactggcgatggccctgacattatcttctgggcacacgaccgctttggtggctacgctcaatctggcctgttggctgaaatcaccccggacaaagcgttccaggacaagctgtatccgtttacctgggatgccgtacgttacaacggcaagctgattgcttacccgatcgctgttgaagcgttatcgctgatttataacaaagatctgctgccgaacccgccaaaaacctgggaagagatcccggcgctggataaagaactgaaagcgaaaggtaagagcgcgctgatgttcaacctgcaagaaccgtacttcacctggccgctgattgctgctgacgggggttatgcgttcaagtatgaaaacggcaagtacgacattaaagacgtgggcgtggataacgctggcgcgaaagcgggtctgaccttcctggttgacctgattaaaaacaaacacatgaatgcagacaccgattactccatcgcagaagctgcctttaataaaggcgaaacagcgatgaccatcaacggcccgtgggcatggtccaacatcgacaccagcaaagtgaattatggtgtaacggtactgccgaccttcaagggtcaaccatccaaaccgttcgttggcgtgctgagcgcaggtattaacgccgccagtccgaacaaagagctggcaaaagagttcctcgaaaactatctgctgactgatgaaggtctggaagcggttaataaagacaaaccgctgggtgccgtagcgctgaagtcttacgaggaagagttggcgaaagatccacgtattgccgccactatggaaaacgcccagaaaggtgaaatcatgccgaacatcccgcagatgtccgctttctggtatgccgtgcgtactgcggtgatcaacgccgccagcggtcgtcagactgtcgatgaagccctgaaagacgcgcagactatggcccaaaaccacgttatcagcttagcttccgccgcagaacgcagggcgcacattgccgataccttcggcaggcacggcatcccgtttcagtttttcgacgcactgatgccgtctgaaaggctggaacaggcaatggcggaactcgtccccggcttgtcggcgcacccctatttgagcggagtggaaaaagcctgctttatgagccacgccgtattgtggaagcaggcattggacgaaggtctgccgtatatcaccgtatttgaggacgacgttttactcggcgaaggtgcggaaaaattccttgccgaagacgcttggctgcaagaacgctttgacccggataccgcctttatcgtccgcttggaaacgatgtttatgcacgtcctgacctcgccctccggcgtggcggattactgcgggcgcgcctttccgctgttggaaagcgaacactgggggacggcgggctatatcatttcccgaaaagcgatgcggtttttcctggacaggtttgccgccctgccgcccgaagggctgcaccccgtcgatctgatgatgttcagcgattttttcgacagggaaggaatgccggtttgccagctcaatcccgccttgtgcgcccaagagctgcattatgccaagtttcacgaccaaaacagcgcattgggcagcctgatcgaacacgaccgcctcctgaaccgcaaacagcaaaggcgcgattcccccgccaacacattcaaacaccgcctgatccgcgccttgaccgatatcagcagggaaagggaaaaacgccggcaaaggcgcgaacagttcattgtgcctttccaataagcggccgcgtcgacacgcaaaaaggccatccgtcaggatggccttctgcttaatttgatgcctggcagtttatggcgggcgtcctgcccgccaccctccgggccgttgcttcgcaacgttcaaatccgctcccggcggatttgtcctactcaggagagcgttcaccgacaaacaacagataaaacgaaaggcccagtctttcgactgagcctttcgttttatttgatgcctggcagttccctactctcgcatggggagaccccacactaccatcatgtatgaatatcctccttagttcctattccgaagggtaatggcatcagggaatggcgaacgcgctccccacactaccatcatgtatgaatatcctccttagttcctattccgaagttcctattctctagaaagtataggaacttcggtggaacgacgcgtaactcacgttaagggattttggtcatgatcagcacgtgttgacaattaatcatcggcatagtatatcggcatagtataatacgacaaggtgaggaactaaaccatggccaagttgaccagtgccgttccggtgctcaccgcgcgcgacgtcgccggagcggtcgagttctggaccgaccggctcgggttctcccgggacttcgtggaggacgacttcgccggtgtggtccgggacgacgtgaccctgttcatcagcgcggtccaggaccaggtggtgccggacaacaccctggcctgggtgtgggtgcgcggcctggacgagctgtacgccgagtggtcggaggtcgtgtccacgaacttccgggacgcctccgggccggccatgaccgagatcggcgagcagccgtgggggcgggagttcgccctgcgcgacccggccggcaactgcgtgcacttcgtggccgaggagcaggactgagtggcagggcggggcgtaaggcgcgccatttaaatgaagttcctattccgaagttcctattctctagaaagtataggaacttcgaagcagctccagcctacacaatcgctcaagacggaacccgcgcttggcaggaaagtaatagggatagcagctccagcctacacaatcgctcaagacgtgtaatgctgcacaataaccctgctgcagaggcctgcatgcaagcttggcgtaatcatggtcatagctgtttcctgtgtgaaattgttatccgctcacaattccacacaacatacgagccggaagcataaagtgtaaagcctggggtgcctaatgagtgagctaactcacattaattgcgttgcgctcactgcccgctttccagtcgggaaacctgtcgtgccagctgcattaatgaatcggccaacgcgcggggagaggcggtttgcgtattgggcgctcttccgcttcctcgctcactgactcgctgcgctcggtcgttcggctgcggcgagcggtatcagctcactcaaaggcggtaatacggttatccacagaatcaggggataacgcaggaaagaacatgtgagcaaaaggccagcaaaaggccaggaaccgtaaaaaggccgcgttgctggcgtttttccataggctccgcccccctgacgagcatcacaaaaatcgacgctcaagtcagaggtggcgaaacccgacaggactataaagataccaggcgtttccccctggaagctccctcgtgcgctctcctgttccgaccctgccgcttaccggatacctgtccgcctttctcccttcgggaagcgtggcgctttctcatagctcacgctgtaggtatctcagttcggtgtaggtcgttcgctccaagctgggctgtgtgcacgaaccccccgttcagcccgaccgctgcgccttatccggtaactatcgtcttgagtccaacccggtaagacacgacttatcgccactggcagcagccactggtaacaggattagcagagcgaggtatgtaggcggtgctacagagttcttgaagtggtggcctaactacggctacactagaagaacagtatttggtatctgcgctctgctgaagccagttaccttcggaaaaagagttggtagctcttgatccggcaaacaaaccaccgctggtagcggtggtttttttgtttgcaagcagcagattacgcgcagaaaaaaaggatctcaagaagatcctttgatcttttctacggggtctgacgctcagtggaacgaaaactcacgttaagggattttggtcatgagattatcaaaaaggatcttcacctagatccttttaaattaaaaatgaagttttaaatcaatctaaagtatatatgagtaaacttggtctgacagttaccaatgcttaatcagtgaggcacctatctcagcgatctgtctatttcgttcatccatagttgcctgactccccgtcgtgtagataactacgatacgggagggcttaccatctggccccagtgctgcaatgataccgcgagacccacgctcaccggctccagatttatcagcaataaaccagccagccggaagggccgagcgcagaagtggtcctgcaactttatccgcctccatccagtctattaattgttgccgggaagctagagtaagtagttcgccagttaatagtttgcgcaacgttgttgccattgctacaggcatcgtggtgtcacgctcgtcgtttggtatggcttcattcagctccggttcccaacgatcaaggcgagttacatgatcccccatgttgtgcaaaaaagcggttagctccttcggtcctccgatcgttgtcagaagtaagttggccgcagtgttatcactcatggttatggcagcactgcataattctcttactgtcatgccatccgtaagatgcttttctgtgactggtgagtactcaaccaagtcattctgagaatagtgtatgcggcgaccgagttgctcttgcccggcgtcaatacgggataataccgcgccacatagcagaactttaaaagtgctcatcattggaaaacgttcttcggggcgaaaactctcaaggatcttaccgctgttgagatccagttcgatgtaacccactcgtgcacccaactgatcttcagcatcttttactttcaccagcgtttctgggtgagcaaaaacaggaaggcaaaatgccgcaaaaaagggaataagggcgacacggaaatgttgaatactcatactcttcctttttcaatattattgaagcatttatcagggttattgtctcatgagcggatacatatttgaatgtatttagaaaaataaacaaataggggttccgcgcacatttccccgaaaagtgccacctgacgtctaagaaaccattattatcatgacattaacctataaaaataggcgtatcacgaggccctttcgtc

SEQ ID NO: 14 - DNA, 6788 bp, Artificial Sequence
  pINT-malE-lex1
tcgcgcgtttcggtgatgacggtgaaaacctctgacacatgcagctcccggagacggtcacagcttgtctgtaagcggatgccgggagcagacaagcccgtcagggcgcgtcagcgggtgttggcgggtgtcggggctggcttaactatgcggcatcagagcagattgtactgagagtgcaccatatgcggtgtgaaataccgcacagatgcgtaaggagaaaataccgcatcaggcgccattcgccattcaggctgcgcaactgttgggaagggcgatcggtgcgggcctcttcgctattacgccagctggcgaaagggggatgtgctgcaaggcgattaagttgggtaacgccagggttttcccagtcacgacgttgtaaaacgacggccagtgaattcgaagatcctttgatcttttctacggggtctgacgctcagtggaacgaaaactcacgttaagggattttggtcatgagattatcaaaaaggatcttcacctagatccttttaaactagtgaagttaccatcacggaaaaaggttatgctgcttttaagacccactttcacatttaagttgtttttctaatccgcatatgatcaattcaaggccgaataagaaggctggctctgcaccttggtgatcaaataattcgatagcttgtcgtaataatggcggcatactatcagtagtaggtgtttccctttcttctttagcgacttgatgctcttgatcttccaatacgcaacctaaagtaaaatgccccactgcgctgagtgcatataatgcattctctagtgaaaaaccttgttggcataaaaaggctaattgattttcgagagtttcatactgtttttctgtaggccgtgtacctaaatgtacttttgctccatcgcgatgacttagtaaagcacatctaaaacttttagcgttattacgtaaaaaatcttgccagctttccccttctaaagggcaaaagtgagtatggtgcctatctaacatctcaatggctaaggcgtcgagcaaagcccgcttattttttacatgccaatacaatgtaggctgctctacacctagcttctgggcgagtttacgggttgttaaaccttcgattccgacctcattaagcagctctaatgcgctgttaatcactttacttttatctaaacgagacatactcttcctttttcaatattattgaagcatttatcagggttattgtctcatgagcggatacatatttgaatgtatttagaaaaataaacaaataggggttccgcgcacatttccccgaaaagtgccacctgaaattggccagatgattaattcctaatttttgttgacactctatcattgatagagttattttaccactccctatcagtgatagagaaaagtgaaatgaatagttcgacaaaaatctagaaataattttgtttaactttaagaaggagatatacaaatgaaaatcgaagaaggtaaactggtaatctggattaacggcgataaaggctataacggtctcgctgaagtcggtaagaaattcgagaaagataccggaattaaagtcaccgttgagcatccggataaactggaagagaaattcccacaggttgcggcaactggcgatggccctgacattatcttctgggcacacgaccgctttggtggctacgctcaatctggcctgttggctgaaatcaccccggacaaagcgttccaggacaagctgtatccgtttacctgggatgccgtacgttacaacggcaagctgattgcttacccgatcgctgttgaagcgttatcgctgatttataacaaagatctgctgccgaacccgccaaaaacctgggaagagatcccggcgctggataaagaactgaaagcgaaaggtaagagcgcgctgatgttcaacctgcaagaaccgtacttcacctggccgctgattgctgctgacgggggttatgcgttcaagtatgaaaacggcaagtacgacattaaagacgtgggcgtggataacgctggcgcgaaagcgggtctgaccttcctggttgacctgattaaaaacaaacacatgaatgcagacaccgattactccatcgcagaagctgcctttaataaaggcgaaacagcgatgaccatcaacggcccgtgggcatggtccaacatcgacaccagcaaagtgaattatggtgtaacggtactgccgaccttcaagggtcaaccatccaaaccgttcgttggcgtgctgagcgcaggtattaacgccgccagtccgaacaaagagctggcaaaagagttcctcgaaaactatctgctgactgatgaaggtctggaagcggttaataaagacaaaccgctgggtgccgtagcgctgaagtcttacgaggaagagttggcgaaagatccacgtattgccgccactatggaaaacgcccagaaaggtgaaatcatgccgaacatcccgcagatgtccgctttctggtatgccgtgcgtactgcggtgatcaacgccgccagcggtcgtcagactgtcgatgaagccctgaaagacgcgcagactatgcacttcattgaaaacaaaaacttcgtcatctccattccgaccgcagacaaacgccgtaatcacatcatccaacagttcggccaaaagaaaattccgtttgaatttttcgatgccttcaccccgagcgaacgtctgaacgaccatctgcagcgctatctgccgaatgtcgcagcaaccccgcgtctgacgatgggtgaaaaaggttgcctgatgtctcactttatgctgtggaaaaaatgtgttgatgacggcctggattacattaccctgtttgaagatgacatcctgctgggtgaaaacgcggaacaattcctggccgaagacgaatggctgaaagtgcgttttaatttccaggaaatctttgttctgcgcctggaaaccttcctgatgccggtgaaaattgaaaaacagcaaggcatcctgccgtttcagcaacgcgaaatcgatatcctgaaatcaaaacatttcggcacggcaggttatgttatttcgcacggtgcagctaaatacctgatcgaagtcttcgaaaaattcagctctgaagaagtgaaaccgattgatgaaatcatgtttaaccagctgattgacatctccggctatcaggtttaccaactgaatccggctatttgcgtccaggaactgcaactgaaccaggaaaatagtgtgctggaatccggtctgcagaaagagcgtaagaaaaacaccgttagccataccaagaaaaccctgaaatatcgtctgacgcgcatgaaagaaaacatcctgcgcgcactgaataaaaagaaatgggaagaacgccaatacatcaaaggtctgcaaggcaaaaatatcatcctgtttatctaggcggccgcgtcgacacgcaaaaaggccatccgtcaggatggccttctgcttaatttgatgcctggcagtttatggcgggcgtcctgcccgccaccctccgggccgttgcttcgcaacgttcaaatccgctcccggcggatttgtcctactcaggagagcgttcaccgacaaacaacagataaaacgaaaggcccagtctttcgactgagcctttcgttttatttgatgcctggcagttccctactctcgcatggggagaccccacactaccatcatgtatgaatatcctccttagttcctattccgaagggtaatggcatcagggaatggcgaacgcgctccccacactaccatcatgtatgaatatcctccttagttcctattccgaagttcctattctctagaaagtataggaacttcggtggaacgacgcgtaactcacgttaagggattttggtcatgatcagcacgtgttgacaattaatcatcggcatagtatatcggcatagtataatacgacaaggtgaggaactaaaccatggccaagttgaccagtgccgttccggtgctcaccgcgcgcgacgtcgccggagcggtcgagttctggaccgaccggctcgggttctcccgggacttcgtggaggacgacttcgccggtgtggtccgggacgacgtgaccctgttcatcagcgcggtccaggaccaggtggtgccggacaacaccctggcctgggtgtgggtgcgcggcctggacgagctgtacgccgagtggtcggaggtcgtgtccacgaacttccgggacgcctccgggccggccatgaccgagatcggcgagcagccgtgggggcgggagttcgccctgcgcgacccggccggcaactgcgtgcacttcgtggccgaggagcaggactgagtggcagggcggggcgtaaggcgcgccatttaaatgaagttcctattccgaagttcctattctctagaaagtataggaacttcgaagcagctccagcctacacaatcgctcaagacggaacccgcgcttggcaggaaagtaatagggatagcagctccagcctacacaatcgctcaagacgtgtaatgctgcacaataaccctgctgcagaggcctgcatgcaagcttggcgtaatcatggtcatagctgtttcctgtgtgaaattgttatccgctcacaattccacacaacatacgagccggaagcataaagtgtaaagcctggggtgcctaatgagtgagctaactcacattaattgcgttgcgctcactgcccgctttccagtcgggaaacctgtcgtgccagctgcattaatgaatcggccaacgcgcggggagaggcggtttgcgtattgggcgctcttccgcttcctcgctcactgactcgctgcgctcggtcgttcggctgcggcgagcggtatcagctcactcaaaggcggtaatacggttatccacagaatcaggggataacgcaggaaagaacatgtgagcaaaaggccagcaaaaggccaggaaccgtaaaaaggccgcgttgctggcgtttttccataggctccgcccccctgacgagcatcacaaaaatcgacgctcaagtcagaggtggcgaaacccgacaggactataaagataccaggcgtttccccctggaagctccctcgtgcgctctcctgttccgaccctgccgcttaccggatacctgtccgcctttctcccttcgggaagcgtggcgctttctcatagctcacgctgtaggtatctcagttcggtgtaggtcgttcgctccaagctgggctgtgtgcacgaaccccccgttcagcccgaccgctgcgccttatccggtaactatcgtcttgagtccaacccggtaagacacgacttatcgccactggcagcagccactggtaacaggattagcagagcgaggtatgtaggcggtgctacagagttcttgaagtggtggcctaactacggctacactagaagaacagtatttggtatctgcgctctgctgaagccagttaccttcggaaaaagagttggtagctcttgatccggcaaacaaaccaccgctggtagcggtggtttttttgtttgcaagcagcagattacgcgcagaaaaaaaggatctcaagaagatcctttgatcttttctacggggtctgacgctcagtggaacgaaaactcacgttaagggattttggtcatgagattatcaaaaaggatcttcacctagatccttttaaattaaaaatgaagttttaaatcaatctaaagtatatatgagtaaacttggtctgacagttaccaatgcttaatcagtgaggcacctatctcagcgatctgtctatttcgttcatccatagttgcctgactccccgtcgtgtagataactacgatacgggagggcttaccatctggccccagtgctgcaatgataccgcgagacccacgctcaccggctccagatttatcagcaataaaccagccagccggaagggccgagcgcagaagtggtcctgcaactttatccgcctccatccagtctattaattgttgccgggaagctagagtaagtagttcgccagttaatagtttgcgcaacgttgttgccattgctacaggcatcgtggtgtcacgctcgtcgtttggtatggcttcattcagctccggttcccaacgatcaaggcgagttacatgatcccccatgttgtgcaaaaaagcggttagctccttcggtcctccgatcgttgtcagaagtaagttggccgcagtgttatcactcatggttatggcagcactgcataattctcttactgtcatgccatccgtaagatgcttttctgtgactggtgagtactcaaccaagtcattctgagaatagtgtatgcggcgaccgagttgctcttgcccggcgtcaatacgggataataccgcgccacatagcagaactttaaaagtgctcatcattggaaaacgttcttcggggcgaaaactctcaaggatcttaccgctgttgagatccagttcgatgtaacccactcgtgcacccaactgatcttcagcatcttttactttcaccagcgtttctgggtgagcaaaaacaggaaggcaaaatgccgcaaaaaagggaataagggcgacacggaaatgttgaatactcatactcttcctttttcaatattattgaagcatttatcagggttattgtctcatgagcggatacatatttgaatgtatttagaaaaataaacaaataggggttccgcgcacatttccccgaaaagtgccacctgacgtctaagaaaccattattatcatgacattaacctataaaaataggcgtatcacgaggccctttcgtc

SEQ ID NO: 15 - DNA, 35 bp, Artificial Sequence
  Primer gal fwd
ttactcagcaataaactgatattccgtcaggctgg

SEQ ID NO: 16 - DNA, 86 bp, Artificial Sequence
  Primer gal rev
ttgataatctcgcgctcttcagcagtcagactttccatatagagcgtaatttccgttaacgtcggtagtgctgaccttgccggagg

SEQ ID NO: 17 - DNA, 58 bp, Artificial Sequence
  Primer ME for
ctgtctcttatacacatctcctgaaattggccagatgattaattcctaatttttgttg

SEQ ID NO: 18 - DNA, 50 bp, Artificial Sequence
  Primer ME rev
ctgtctcttatacacatctcagcattacacgtcttgagcgattgtgtagg

SEQ ID NO: 19 - DNA, 30 bp, Artificial Sequence
  Primer galE_NdeI-for
gatcacatatgagagttctggttaccggtg

SEQ ID NO: 20 - DNA, 40 bp, Artificial Sequence
  Primer galE_XhoI-rev
gatcactcgagtcattaatcgggatatccctgtggatggc

SEQ ID NO: 21 - DNA, 35 bp, Artificial Sequence; identical to SEQ ID NO: 15
  Primer gal fwd

SEQ ID NO: 22 - DNA, 83 bp, Artificial Sequence
  Primer gal rev
ttgtaatctcgcgctcttcacatcagactttccatatagagcgtaatttccgttaacgtcggtagtgctgaccttgccggagg

SEQ ID NO: 23 - DNA, 54 bp, Artificial Sequence
  Primer ME for
ctgtctcttatcacatctcctgaaatggccagatgtaattcctaatttttgttg

SEQ ID NO: 24 - DNA, 44 bp, Artificial Sequence
  Primer ME rev
ctgtctcttatcacatctcacattacatctgagcgattgttagg

SEQ ID NO: 25 - DNA, 30 bp, Artificial Sequence; identical to SEQ ID NO: 19
  Primer galE_NdeI-for

SEQ ID NO: 26 - DNA, 40 bp, Artificial Sequence; identical to SEQ ID NO: 20
  Primer galE_XhoI-rev

SEQ ID NO: 27 - DNA, 60 bp, Artificial Sequence
  Primer lex1 pINT-f
gtcgatgaagccctgaaagacgcgcagactatgcacttcattgaaaacaaaaacttcgtc

SEQ ID NO: 28 - DNA, 60 bp, Artificial Sequence
  Primer lex1 pINT-r
gatggcctttttgcgtgtcgacgcggccgcctagataaacaggatgatatttttgccttg

SEQ ID NO: 29 - DNA, 60 bp, Artificial Sequence
  Primer pINT lex1-f
caaggcaaaaatatcatcctgtttatctaggcggccgcgtcgacacgcaaaaaggccatc

SEQ ID NO: 30 - DNA, 60 bp, Artificial Sequence
  Primer pINT lex1-r
gacgaagtttttgttttcaatgaagtgcatagtctgcgcgtctttcagggcttcatcgac

SEQ ID NO: 31 - DNA, 60 bp, Artificial Sequence
  Primer lgtB pINT-f
gtcgatgaagccctgaaagacgcgcagactatggcccaaaaccacgttatcagcttagct

SEQ ID NO: 32 - DNA, 60 bp, Artificial Sequence
  Primer lgtB pINT-r
gatggcctttttgcgtgtcgacgcggccgcttattggaaaggcacaatgaactgttcgcg

SEQ ID NO: 33 - DNA, 60 bp, Artificial Sequence
  Primer pINT lgtB-f
cgcgaacagttcattgtgcctttccaataagcggccgcgtcgacacgcaaaaaggccatc

SEQ ID NO: 34 - DNA, 60 bp, Artificial Sequence
  Primer pINT lgtB-r
agctaagctgataacgtggttttgggccatagtctgcgcgtctttcagggcttcatcgac